European Patent Application EP 4 640 828 A1, published October 29, 2025. Title: Antigen peptide with multiple KRAS variant peptide linked together, nucleic acid encoding same, and use thereof. Applicant: HANMI PHARM. CO., LTD. The sequence listing filed with the application follows.

SEQUENCE LISTING (557 sequences)

SEQ ID NO: 1 - RNA, 411 nt, synthetic construct
  source 1..411: mol_type = other RNA
atgacagagtacaagctggtggtcgtgggggccaggggcgtgggcaagagcgccctgactatccagctggaatacaagctggtggtggtgggcgccgacggcgtggggaagtccgccctcacaatcgagtacaagctggtcgtggtgggggccgtgggcgtcgggaagtccgccctgacaatcgagtacaagttggtggtggtgggcgcctgcggggtgggcaagagcgccctgaccatctacaagctcgtggtggtgggggccggggacgtggggaagagtgccctgaccatccagtataagctggtggtggtcggcgccgggtgcgtgggcaagtccgccctgacaatccagctgctggatatcctggataccgccggccacgaggagtacagcgccatgagggatcag

SEQ ID NO: 2 - RNA, 357 nt, synthetic construct
  source 1..357: mol_type = other RNA
tacaagctggtcgtcgtgggggcctgcggcgtggggaagtccgctctgacctacaaactggtggtggtgggggccgatggggtgggcaagtccgccctgacctacaagctggtggtggtcggggccgtcggcgtgggcaaaagcgccctgacatacaagctcgtggtggtgggcgccaggggggtgggcaagtccgccctgacaaagctggtcgtggtgggcgccgggtgcgtgggcaagagcgccctgacaatcaagctggtggtggtgggggccggggatgtgggcaagagcgccctgaccatcctggacatcctggacacagccgggcacgaggagtacagcgccatgagggat

SEQ ID NO: 3 - RNA, 501 nt, synthetic construct
  source 1..501: mol_type = other RNA
ctgctgagcgtgggggggtacaagctcgtggtggtgggcgcctgcggcgtggggaagtccgccctgacactgctgtccgtgggcggctacaagctggtggtcgtgggcgccgacggggtgggcaagagcgccctcaccctgctcagcgtggggggctacaagctggtcgtggtcggggccgtgggcgtgggcaagtccgctctgacactgctgtccgtgggcgggtacaagctggtggtggtgggggccaggggggtcgggaaatccgccctgactctgctgagcgtcggcggcaagctcgtggtggtgggggccgggtgcgtggggaagtccgccctgacaattctgctgagcgtgggcgggaagctggtcgtggtgggcgccggggatgtgggcaagagcgccctgaccatcctgctgagcgtcggcggcctggacatcctggacaccgccggccacgaggagtacagcgccatgagggatctgctcagcgtggggggg

SEQ ID NO: 4 - RNA, 252 nt, synthetic construct
  source 1..252: mol_type = other RNA
gttggagcctgtggagttggtaaaagtctcctaagcgttggaggagtagttgtgggagcttgtggagtaggtctgttaagcgtgggtggtgtaggagcttgtggagtaggaaagtctctgctctccgtaggaggagtagtagtaggagcatgcggagtcggactgctgtccgtaggaggtgtaggagcatgcggagtaggaaagtcacttctgtctgtaggaggagtagtagtaggagcttgtggagtagga

SEQ ID NO: 5 - RNA, 252 nt, synthetic construct
  source 1..252: mol_type = other RNA
gtgggcgcctgtggagtaggaaaatctctcttatctgttggaggagtggtggtcggagcatgcggagtaggactcttgtccgtaggaggtgtgggagctgacggcgtgggtaaatccctattaagtgtcggaggagtggtcgtgggagctgacggtgttggtttattgagcgttggaggaggagcgggagatgttggaaagtcagccttacttagcgtcggaggagttgtgggggctggtgacgtgggaaag

SEQ ID NO: 6 - RNA, 441 nt, synthetic construct
  source 1..441: mol_type = other RNA
atgacagaatacaaacttgtggtagttggagcatgcggtgtgggtaagagtgccctcaccatccaactaattcagaaccacttcgttgacgaactcctctcagtggggggggttggagcatgtggtgtagggaagctgttgagcgtcggcgggatgactgaatacaaacttgtggttgttggagcagatggggtcggaaaatccgccttgacaatacagcttattcagaatcactttgtggatgagctgttaagcgttggcggcgtcggagctgatggcgtcggaaagctcttgtctgtgggcggcactgagtataaattagtggtagtcggggctggagacgtgggcaagagtgcccttaccatccagctcatccagaatcattttgtggacgagtatctattgtccgtgggaggtggagctggtgacgtcggaaagtct

SEQ ID NO: 7 - RNA, 648 nt, synthetic construct
  source 1..648: mol_type = other RNA
atgactgaatataaactcgtcgtggttggagcaggttgcgttggcaaaagcgcccttacaatccagctgatacagaaccacttcgtggatgagttattgagcgtcggcggcatgacagagtacaagttggtggtggtgggcgcctgtggggtggggaaatctgcccttactatccagctgatccagaaccactttgtggatgagttacttagcgtcggagggatgacagaatacaaactggtcgtggtcggcgctgatggcgttgggaagagtgctctgacaattcaactcatccagaatcacttcgtagacgaactgctttcagtcggggggatgacggagtataagctcgttgtggtaggcgccggagacgtaggcaagtccgcactgaccattcagctcattcaaaatcattttgtagacgaactattgtctgtgggcggtatgaccgagtacaagctggttgttgtgggtgccgtgggggtgggtaagtcagccctcaccattcagctcatccaaaaccatttcgtggacgagctgctgagtgtcggaggtacctgcctcctggacatattggacactgcggggcatgaggagtattccgcaatgcgcgatcagtacatgaggaccggagaaggatttctgtgc

SEQ ID NO: 8 - RNA, 351 nt, synthetic construct
  source 1..351: mol_type = other RNA
atgacagagtataagctggtcgtggtcggcgcgtgcggagtggggaaatcagctctcaccattcagctaatccagaaccacttcgttgacgaagtcggcgcttgcggtgtcggaaagatgacggagtataaacttgtcgtagttggcgccgacggtgttggaaaatccgcattaaccatacaattgatccagaaccacttcgtggacgaagtgggggctgacggcgtaggaaaaacagagtacaagctggtggtggttggcgcaggggatgtgggtaagagcgccctgactattcagctgatccaaaatcattttgtggatgaatacggagcaggcgatgtggggaagtct

SEQ ID NO: 9 - RNA, 1179 nt, synthetic construct
  source 1..1179: mol_type = other RNA
tgtataaacctcgattgggatgtaatccgcgacaaaaccaagacaaaaattgaatctctcaaggagcacggccctatcaaaaataaaatgtcagagtcacccaataagacggtgtctgaggaaaaggccaagcaatacttggaagaatttcatcaaaccgccttggaacatccggaactaagcgagcttaagacagttacaggtactaacccagtgtttgccggagctaactacgccgcgtgggcggtcaatgtagcccaggtcattgatagtgaaactgctgacaatttagaaaagacaactgccgctctctccattctgcccggaatagggagcgttatgggtatcgcagatggcgcggtgcatcataacaccgaggagatcgtcgcacagtcgatcgctctcagtagcctaatggtggctcaggcaattcctctggtcggggaactggttgacatcggattcgccgcatacaatttcgtagagtctattataaatcttttccaggtggtccacaactcatataatcgaatgactgagtacaagctggtagtggtaggggctggatgcgtcgggaagtcagccctgactatacagctgatccagaaccacttcgtggatgagctcctatccgtgggcgggatgacggaatataagctcgttgtggtaggggcttgtggagtgggcaagtccgcactgacaatccagctgatccagaatcactttgtggatgagctcctgagtgtggggggaatgaccgaatacaaacttgttgtggtgggcgctgacggagttggtaaaagcgcccttaccatccaactgattcagaaccactttgtcgacgagttactgagcgtcggagggatgaccgagtataaattggtggtggtgggcgctggcgacgtgggcaaaagtgcactgacaattcagctgattcagaaccactttgtggacgagttgctaagcgtcggtggaatgaccgagtataagttggtggttgtcggcgcggttggtgtgggaaaatctgcccttacaatccagctgattcaaaaccatttcgtcgacgagctgctgtccgttgggggcacgtgcttgctcgacatcctggatactgccggccacgaagagtactccgccatgcgggatcaatatatgcgtaccggcgaggggttcttatgt

SEQ ID NO: 10 - RNA, 1197 nt, synthetic construct
  source 1..1197: mol_type = other RNA
atgacagagtacaagctggtggtcgtcggagccggttgcgtaggaaagagcgcattaaccatccagctaatccaaaaccatttcgtggacgaactcctgtcagtggggggaatgactgaatacaagttagtggtggttggggcctgtggtgtgggaaaatccgctctcacgatccagctgattcagaaccacttcgtcgacgagttactttccgttggaggcatgaccgaatataaactggttgtcgtgggggctgatggagttggcaagtctgccttgactattcaactgatccagaatcattttgtggatgagctcctgagcgtaggggggatgacagagtataaactcgtcgtggtgggtgccggagatgttgggaaatctgctcttaccatacagttaatccaaaatcacttcgttgatgaactgctttcagtgggcggaatgactgagtacaagttggtggtggtgggggctgtgggggtgggaaagtctgcactgactattcagctcattcagaaccacttcgtggatgagctgctctcggtaggcgggacctgtctgctagacattctggacacggccggccatgaggagtatagcgcaatgagagaccaatacatgcggaccggcgaaggctttctttgcctgctcagcgtgggcggctgtataaacctcgactgggatgtgatccgcgataaaaccaagaccaagatcgaaagcctaaaggagcatggccctattaagaataaaatgtcagaatctcccaataaaacagtatccgaggaaaaggccaaacagtatttggaagagtttcaccagaccgccctggaacacccagagctgtccgaactgaagacagtcactgggacaaatcctgtcttcgccggtgctaactacgcggcatgggcggtcaatgtagcccaagttatcgatagtgagactgccgacaaccttgagaaaaccacagcagcattgagcatattgccgggcatcggttctgtcatgggcatagctgacggcgctgtgcaccacaacacagaggagatcgtcgctcagagtattgcgctgtccagtcttatggtggcccaggccatcccacttgttggtgaactggtggacatcggatttgcagcgtacaactttgtcgagtcaattattaatctgttccaggttgtccataacagttataatcgt

SEQ ID NO: 11 - RNA, 1155 nt, synthetic construct
  source 1..1155: mol_type = other RNA
tgtataaatcttgactgggacgtcattagggataagacaaagaccaagatagagtccttgaaggagcacggccccatcaaaaacaaaatgtcggagagcccaaacaaaacagtgagtgaagagaaagcaaagcagtatcttgaagagtttcaccagacggctctggaacatcctgagctgtctgaacttaagacagtgaccggcacaaaccctgtgtttgcaggagctaattatgcggcttgggccgttaacgtggctcagatgactgagtataaactggttgtggtgggcgccggctgcgtcggaaagagcgcgctgaccattcaacttattcaaaatcacttcgttgatgaactcctgtcagtaggaggcatgactgaatataagttagtggtcgtgggcgcctgtggggtgggtaaaagcgccctaactatacagctaatccagaaccactttgtagacgagcttctgtccgtggggggtatgacagagtacaagctggtggttgtaggtgcagacggcgtcggcaaatccgccctcactatccagctgattcagaaccactttgtagacgagttgctctcagtcggaggaatgactgaatacaaacttgttgtggttggggctggggatgtcggaaagagtgctctgacgattcagctgatccagaaccattttgtggacgaactcctgtcagttgggggcatgaccgagtacaagctggtggttgtgggagcggtcggggtcgggaagtccgccttaacaatccagctgatccaaaatcacttcgtggatgaactgttgtcagtggggggcacctgcctgctcgacatcctcgataccgccggtcacgaagagtactccgccatgcgtgatcaatatatgcgaacgggggagggtttcttatgcaatttggagaaaaccaccgcagcactatctatcctgccgggaataggtagcgtcatgggcatcgccgacggagcagtacatcataatactgaagaaattgtggcccaatctatcgccttaagttctttgatggtggctcaggctattcccctggtcggggagctggtagatattggcttcgctgcctacaacttcgtggagagcatcattaatttgttccaggtcgtgcataatagctacaacagg

SEQ ID NO: 12 - RNA, 408 nt, synthetic construct
  source 1..408: mol_type = other RNA
tacaagctagtggtggtcggcgcatgcggcgtgggaaagagcgcgctaacctataaattggtcgttgtgggcgccgatggtgtagggaaatctgcgctgacctacaagctcgtggtggtgggggcagtcggcgtcggcaaaagtgccctgacttataagctggtcgtggtaggtgctcgtggcgttggaaagtccgccttgacaaagctggttgtcgtgggggccggatgcgtgggcaaatctgctcttacaatcaaattagtagttgtgggagctggagacgtaggtaaatccgcactgacgatactcgatattctcgacaccgctggacacgaagagtacagcgccatgcgcgacaagctggtcgtggtgggggccggcagagttggtaagtcagcactcactatc

SEQ ID NO: 13 - RNA, 1206 nt, synthetic construct
  source 1..1206: mol_type = other RNA
atgaccgagtacaaactcgttgtggtgggggcctgcggagtgggcaagtctgcattgaccatacagttgatccagaatcatttcgtggatgagctcctaagtgtcggcggcgtcggagcgtgtggcgtgggcaaactcctcagcgtggggggcatgactgagtataagttagtagtcgttggtgccgatggagtaggcaaatcggcgttaacgatccagcttattcagaatcatttcgtagatgagttgctgtccgttggcggagtcggggccgacggcgtgggcaaattgcttagtgtgggggggatgaccgagtataagttagtcgtcgtgggtgctgtgggcgtaggtaaatccgccctgactatacagcttattcaaaaccattttgtggatgagttgctgtctgtaggaggagtgggagctgtgggcgttgggaaattgctgagtgtgggagggatgactgagtacaagctggtggtcgtcggtgcccggggcgttggtaagagcgccctgaccatacaactcattcagaaccactttgtagacgaactgctaagcgtggggggcgtgggagcaaggggagtcgggaaactcctcagcgtggggggtacagaatacaagctggttgtagtcggcgccggttgtgtcgggaagtccgcactcacaattcagcttatccagaatcacttcgtggacgagtatctgttgtcagtgggcggtggggcaggctgcgttggaaagagcctgctctcagtgggcggcacagagtacaaattagtggtcgtgggagctggggacgtgggaaagtccgctctcactatccagctgattcagaaccattttgtcgacgaatatctcctgtcagtggggggcggggctggggacgtgggcaaatcacttctaagcgtgggcggaacctgcctgctggatatcctggacacagcgggacacgaagaatacagcgccatgagagatcagtacatgcgaacgggtgaaggcttcctgtgcctcctgtctgttggtggcacagcagggcacgaggaatactccctgctgtccgtgggtgggactgaatataagctggtagttgttggcgcaggaagagttgggaagagtgctctaaccatccaacttatccagaaccactttgtggacgagtatctgctttctgttggtggcggcgccgggcgcgtcggaaagtct

SEQ ID NO: 14 - RNA, 936 nt, synthetic construct
  source 1..936: mol_type = other RNA
atgacagaatacaagttagtggtggtaggagcgtgtggagtggggaaaagcgccctaactattcagttgatacaaaaccatttcgtggacgaagtgggcgcatgtggagtcggcaagatgaccgagtataagctcgtagtcgtgggggccgacggcgtggggaaatcagcccttactatccagcttatacaaaaccattttgttgacgaagtaggcgccgacggggtcggaaagatgaccgagtacaagctggttgtcgtcggggccgtaggggttggcaaaagcgccctgactatccagctcatccaaaatcatttcgtcgacgaggtgggcgccgttggagtcggtaaaatgacggaatacaagttggtggtagtgggggctcggggggtgggcaagagtgctttgaccatacagttaattcagaaccactttgtggatgaggtcggcgctcgcggagtcggcaaaaccgagtataaattggttgttgtcggcgcaggctgtgtgggcaagtctgctctcaccattcaactaatccagaaccactttgttgatgagtacggagcaggctgcgtgggaaaaagcacggagtacaagctggttgtcgtaggagcaggagacgtgggcaaatccgctctgacaattcagcttatccagaatcactttgtggatgaatatggtgccggggatgtcggtaaaagtacctgcttactggacatcctggacactgctggtcacgaggaatactccgcgatgcgagatcagtatatgcggacaggagagggtttcctgtgcacagcaggccatgaggaatattctactgaatataagctggtggtggtgggggctggtagagtggggaagtcagcactgacaatccagctcattcagaatcacttcgttgatgagtacggtgcgggtagagtgggcaagtcc

SEQ ID NO: 15 - RNA, 1206 nt, synthetic construct
  source 1..1206: mol_type = other RNA
atgacggaatacaagctcgtcgtggtgggcgccgatggcgtcggcaagtcggcactgactatccagctcatacaaaatcattttgttgatgaacttttatccgtcggtggagtgggggcggacggagtggggaagctgctgagcgttggtgggatgaccgaatacaaactggtggtggtcggggcgtgtggggtgggcaaatcagccctcacaatacagctgattcagaaccactttgttgacgagcttctgtccgtgggcggggtgggggcatgtggagtggggaagctcctgtccgtagggggcatgactgagtacaagctggttgttgtaggtgctgttggagtgggaaagagcgccctcacaatccaattgatccagaatcacttcgtcgacgagctcttgagcgttggaggtgtgggggccgtaggcgtgggcaagctgctatctgtgggtggaatgaccgaatataagttggtagtggtgggggctcgcggagtcgggaagagtgctcttactattcagctgattcagaaccatttcgtagatgaactcctatcagtcggtggcgtgggcgccagaggcgtgggcaaactgttatcagtgggcggtactgagtacaaactagtagtcgtaggagctgggtgtgtgggcaaaagtgcactcaccatccagctgatccagaaccatttcgtggatgagtatttgttgagtgtcggaggtggagctggctgcgtgggcaaaagcctgctgtccgttggggggacggaatacaaactagttgttgtgggggctggtgatgtcggaaagtccgccttgactattcagcttattcaaaatcactttgtcgacgagtatcttctgagcgtcggcggcggcgcaggtgacgtaggaaagtctttactgtcagttgggggaacctgccttctggacatcctggacacagccggccacgaggaatacagcgccatgcgggatcagtatatgaggacaggagaaggcttcctctgcctcttaagtgtcggcggtacagctggccacgaggagtattctctgctgtctgtcggaggcaccgagtacaaacttgtggtggttggagcagggcgtgtcggcaaatctgccctgaccatccagctgatacaaaaccattttgtggatgagtatttactttccgtgggaggcggtgcgggacgagtgggcaagagc

SEQ ID NO: 16 - RNA, 1224 nt, synthetic construct
  source 1..1224: mol_type = other RNA
tataagttggtggtggttggggcatgtggcgtaggtaagagcgcactgacttataagctagttgtcgtgggagctgacggagtggggaagagtgcactcacatacaagctcgtcgtggtgggcgccgtcggcgtagggaaatcagctcttacctataaactcgtggtggtgggcgctcgcggtgtgggcaaaagtgccctgaccaagctggtcgtcgtgggcgccggctgcgttgggaaatccgccctgacaatcaaattggtcgtcgtgggcgccggggacgtgggtaagtcagccttgaccatcctcgacatactggacactgccggccacgaagaatattctgccatgagggataaattagtggtggtaggtgccggtagagtggggaagtcggctctcaccatttacaagctggtggtagtcggcgcatgtggagtgggaaaaagcgccctgacatacaaattagtggtggtcggtgctgatggggtcggcaagtcagctctgacctacaaactcgttgtcgttggggccgtcggagtgggtaaatccgccctgacctataaattggtcgtggtaggggctcggggagtcgggaaatctgcgctgaccaagctcgttgtggtgggagcaggttgcgttggtaagtctgctttgactatcctcgacatcctcgacaccgcaggacatgaggagtactccgccatgcgtgacaagctagtagttgtaggagccggtgatgtgggaaagtccgctctgacaattaaattggtagtcgtgggggccggcagagtgggaaaaagcgcgctgacaatctataaacttgttgtggtgggcgcagtcggagttggtaagtcagctctgacttacaagctcgttgttgtgggcgctcgcggggtgggcaagtctgccctaacaaaactagtggtggtcggcgccgggtgcgtaggaaagagtgctctgaccatacttgacattctggatactgcgggccacgaggaatatagcgcgatgcgagattacaaactggttgttgtgggagcatgtggcgtcgggaagtccgcattaacgtacaagttagtggtggtcggagcggatggcgttgggaagtctgcacttacgaagttggtggtggtgggggccggagacgtaggcaagtccgcacttaccatcaaactggttgtcgtcggcgccgggcgggtgggcaagagcgcactgactatt

SEQ ID NO: 17 - RNA, 1053 nt, synthetic construct
  source 1..1053: mol_type = other RNA
atgacggaatacaagctcgtcgtggtgggcgccgatggcgtcggcaagtcggcactgactatccagctcatacaaaatcattttgttgatgaacttttatccgtcggtggagtgggggcggacggagtggggaagctgctgagcgttggtgggatgaccgaatacaaactggtggtggtcggggcgtgtggggtgggcaaatcagccctcacaatacagctgattcagaaccactttgttgacgagcttctgtccgtgggcggggtgggggcatgtggagtggggaagctcctgtccgtagggggcatgactgagtacaagctggttgttgtaggtgctgttggagtgggaaagagcgccctcacaatccaattgatccagaatcacttcgtcgacgagctcttgagcgttggaggtgtgggggccgtaggcgtgggcaagctgctatctgtgggtggaatgaccgaatataagttggtagtggtgggggctcgcggagtcgggaagagtgctcttactattcagctgattcagaaccatttcgtagatgaactcctatcagtcggtggcgtgggcgccagaggcgtgggcaaactgttatcagtgggcggtactgagtacaaactagtagtcgtaggagctgggtgtgtgggcaaaagtgcactcaccatccagctgatccagaaccatttcgtggatgagtatttgttgagtgtcggaggtggagctggctgcgtgggcaaaagcctgctgtccgttggggggacggaatacaaactagttgttgtgggggctggtgatgtcggaaagtccgccttgactattcagcttattcaaaatcactttgtcgacgagtatcttctgagcgtcggcggcggcgcaggtgacgtaggaaagtctttactgtcagttgggggaacctgccttctggacatcctggacacagccggccacgaggaatacagcgccatgcgggatcagtatatgaggacaggagaaggcttcctctgcctcttaagtgtcggcggtacagctggccacgaggagtattct

SEQ ID NO: 18 - RNA, 1665 nt, synthetic construct
  source 1..1665: mol_type = other RNA
atgacagagtataaactcgtggtggtcggcgcagatggcgttggaaagagcgccctgactattcagctcatccagaaccatttcgtagacgaactcctgtctgtaggaggagtcggcgcagacggtgtgggaaagctgctgtctgtgggcggtatgaccgaatacaagttagtggtggtcggggcctgcggtgtgggtaaaagcgctctgaccatacagcttatccagaaccacttcgtggatgagctcctgtctgttgggggagtgggggcttgcggagttggcaagctgctttcagtgggcgggatgacagaatataaattggtggtagtgggggccgtaggcgtcggcaagagcgccctgactatacaactgatccaaaaccacttcgtggacgagttgctctccgtgggtggcgtgggcgccgttggagtcgggaaactcctgtccgtcggtggcatgactgagtataaacttgttgtagtcggggcacggggcgtgggaaagtccgctttaaccatacaattgatacagaaccactttgttgatgaactgctgtctgtgggtggggtgggtgccaggggagtcggtaagctgttgtcagtaggagggacctgtctcctagacattctggacacagccggccacgaggagtactcagctatgcgcgatcagtatatgagaacaggggagggatttctgtgtctcctctccgtcggagggacagcagggcacgaagagtacagcctgctttcggtggggggcactgagtacaagctagtcgtggttggcgcaggcgacgtgggtaaatctgccctcaccattcagttaattcagaatcatttcgtcgatgaatatctgctgagtgttggcggcggcgctggagacgtcggcaaatcccttctgagcgtcgggggaatgacggagtataaactggtagtcgtaggtgctgccggcgtcggcaaaagcgcgctaaccatccagctgatccagaatcactttgtggatgaattgttgagtgttgggggggtgggagccgctggagtggggaagttactaagtgtcggtggcagatcttacggaatccctttcatcgaaacctcaaccaagactcgtcaaagggttgaagacgctttctatacacttgtcagagagattaggcagttgctttccgtgggtggagaaacctccacaaagacgcggcaactcctcagtgtcgggggcactgagtacaagctggtggtagtgggagccggttgcgtgggcaagtcagcgctgacaatccagctcatccagaatcattttgttgatgagtacttgttatcagttggcggaggcgcaggctgcgtggggaaatcgcttctgtccgttggaggtatgactgagtacaagctggtggtggtgggggcgtctggggtggggaaatctgcactgacgattcaactgatccagaatcattttgtagacgagttactgagtgtgggaggcgtgggcgcgtccggcgtgggtaagttgctaagcgtgggggggacctgtttgctggatattctggacactgccggacgagaagaatacagtgcaatgagggatcagtatatgcgaaccggagagggctttctttgtctgctcagcgtcggcggaacagccggccgcgaagagtacagc

SEQ ID NO: 19 - RNA, 1206 nt, synthetic construct
  source 1..1206: mol_type = other RNA
atgacggaatataagctcgtggtcgttggggcctgtggcgtgggtaagagcgcactaaccattcagttaatccagaaccactttgttgatgaacttctcagcgtgggcggtgttggggcctgcggcgttggaaaactgttgtccgtgggtggcatgacagagtacaaactggtcgtggtgggggctgtgggtgtgggcaagtccgccctgactatccaactgatacagaaccatttcgtagatgaactgttgagtgtgggcggagtcggcgcagtcggggtaggtaaattgctgagcgtgggaggcatgactgagtataaactcgtggttgtgggtgcagatggagtaggaaagagtgccctcacaatacaactgattcagaatcattttgtcgatgaactgctgagcgtcggcggagtgggagctgatggtgttggcaagctgctttcagtagggggaacctgcctgctggacatcctggacaccgcggggcacgaagagtatagcgctatgcgggaccagtacatgagaaccggtgagggctttctgtgtctgctgtctgtcggaggaacagccggccacgaggagtattctctactatcagtaggcgggactgagtacaagctggtggtggttggcgctggctgtgtggggaaatctgcattaacgattcaactgatccagaatcacttcgtcgatgagtacctcctctcagtcggcggaggcgcaggctgcgtgggcaagtcactcttaagcgtgggcggcacagagtacaagctggttgtcgttggggcaggggacgtcgggaagtccgccctgactatccagctgattcagaaccattttgtggacgaatatctgctgtccgtcggggggggtgctggagacgtgggaaaatccttgctcagtgtaggaggaatgacagagtacaaacttgtggtggttggcgctgctggagtaggaaaatccgccctgaccatacaacttattcagaatcacttcgtggacgagttgctcagtgtagggggtgtcggggcggccggggtggggaagttgctttcggttgggggtatgactgaatacaagttggtggtggtgggcgcgagcggggtgggtaagtctgccttgaccatccagctgatccagaaccatttcgttgatgaacttctttctgtgggaggagtcggcgcctcgggcgtggggaaa

SEQ ID NO: 20 - RNA, 1206 nt, synthetic construct
  source 1..1206: mol_type = other RNA
atgacagagtacaaactggtagtagtgggagcagatggggttggcaaatccgcgctcaccatccagctgattcaaaaccatttcgtcgatgagctgctgagcgttgggggagtgggcgctgacggggtgggcaagctcctttctgtaggcggaatgaccgagtataaactcgtagtggtcggagctgtgggagtgggaaagtcagcgctcactatccaactaatacagaatcactttgtcgacgaactgctttctgtcggtggagtgggcgccgtgggtgtcggcaagctgcttagcgtggggggaatgacagaatacaagttggtcgttgttggtgcccgcggagtgggcaaatctgcactgaccatccaactgatccagaaccactttgtggatgagctactttccgtgggaggcgtcggtgccaggggtgtgggaaagctcctgagtgttggtggcacatgtttgttagacattctcgacacggctgggcatgaggagtatagcgctatgcgggatcagtatatgagaaccggcgaaggctttctctgccttctctcagtgggcggcacagccgggcacgaggaatattccctgctttcggtgggggggacttgcttgctggacatattagacacagcagggagggaagagtattccgcaatgcgagatcagtacatgcgtactggggaagggttcctgtgcctgctgagtgtgggaggcaccgccgggagggaggaatacagccttctgtcagtcggcggcactgagtacaagctggttgtggtgggagccggatgtgtcggtaaaagtgccctaaccatccagctcattcagaaccacttcgtcgatgagtatttgctgtccgtaggcggcggggccggctgtgttgggaaaagcctgctgagcgtaggagggatgactgagtacaagctcgttgtcgtgggtgcatgcggagtagggaagtcagcgctgacaattcagttaatccagaatcacttcgtcgatgaacttctaagtgtgggtggagtcggcgcctgtggagtgggtaagttgctctccgttggaggcacggagtacaagctggtcgtggttggcgccggcgacgtgggcaaaagcgctttgaccattcaactgatccagaatcattttgtggatgaatacttgctctctgtgggtggcggggcaggggacgtggggaaatct

SEQ ID NO: 21 - RNA, 1206 nt, synthetic construct
  source 1..1206: mol_type = other RNA
atgactgaatataaattagttgtggtgggagccgatggagtggggaaatccgcgttgacaatccagctgatccagaaccattttgttgacgaactcctctcagtcgggggcgttggagctgatggcgttggcaagctgctgtctgtggggggaatgacggaatacaagctggtcgtcgtgggcgcggtcggggtaggtaagtccgcgctgacaattcagctgattcagaatcacttcgtggatgagctgctgagcgtaggcggcgtgggcgccgtgggagtcggtaagttgctgtctgtgggtggtaccgagtacaagctcgtggttgtcggtgctggtgacgtgggcaagtcggctctgacgatccaactgatccagaatcatttcgttgatgagtaccttctgagcgtagggggcggggccggagatgtcggcaaatctctcctcagcgttggcgggaggtcatacgggatacctttcattgagacttccaccaaaactcgtcaacgcgtcgaggatgccttttataccctagtgagagagatccgacagctgctgagtgtgggcggtgaaacaagcaccaagacccggcagttactttctgtggggggcatgacagaatacaagttggtagttgtcggcgcctgcggggtggggaaaagtgctctaaccattcaattaatccaaaatcactttgtcgacgagctccttagtgtcggaggcgtgggcgcctgcggggtaggcaaactcctttcagtcggcggaatgaccgaatataaactggtggtggtgggagctgcaggagttggaaaaagcgctctgactatccaactgattcagaaccatttcgtggacgagctgctcagtgtggggggtgtcggggcagccggcgtgggaaaacttctgagcgtgggcgggatgaccgaatacaagctggtggtggttggcgcatccggtgtgggaaagtcagccctgacaatccagcttatacagaaccacttcgtcgacgaacttttgtctgttgggggtgtgggcgcatctggagtcggaaagctactatcggttggaggtacagagtataaattggtggtggtaggtgctggatgtgtcggcaagtccgcacttactatacagctcattcagaaccactttgtagacgagtatttactcagcgtgggcgggggggcagggtgcgtaggcaagtcc

SEQ ID NO: 22 - RNA, 1053 nt, synthetic construct
  source 1..1053: mol_type = other RNA
atgacggaatataagttggtcatggtgggtgcggatggtgtaggcaaatcagctctgactatccaactgatccagaatcactttgtggacgaactgttatcagttgggggggtcggggctgacggtgtcggaaaactgctaagtgtcggcggcatgaccgaatataagctcgttgtggtgggggcttgtggagttggcaagtccgctctgactatccaactaattcagaatcatttcgtcgatgagctgctgagcgttggaggagtcggcgcttgcggagtaggcaaacttctgtcagtgggaggcatgaccgaatacaagctcgtggtggtaggcgccgttggtgtagggaagagtgcgctaaccattcaacttatccagaaccattttgttgacgagcttctctccgtcggtggtgtaggcgcggtgggagtgggcaagctgctctccgtcggcggcatgaccgagtataaacttgtagtggtgggcgccaggggcgtggggaaaagcgccctgacaatccagctcatacagaatcacttcgtagacgagctgctgagtgttggaggagtgggcgcccgcggcgttggtaagctgctcagcgtgggggggactgaatataaactcgtcgtcgtgggagcaggctgtgtggggaagagtgccttgaccattcagttgatccagaaccacttcgtcgacgagtatctgttgtctgtgggaggcggagcagggtgcgttggaaagagccttctctctgtgggtggcacagaatacaaactggttgtcgtgggggccggcgacgtgggcaagagcgccttgactattcaactcatacagaaccactttgtggatgagtaccttctctctgtcgggggaggcgccggggacgtggggaaaagcctcctgtcggtgggaggaacgtgtcttctggatattttagacaccgcagggcatgaggagtactccgcaatgcgagatcagtacatgaggacaggtgagggtttcctgtgcttgctgtccgtgggaggtacagccggccacgaggaatactct

SEQ ID NO: 23 - protein, 137 aa, synthetic construct
MTEYKLVVVGARGVGKSALTIQLEYKLVVVGADGVGKSALTIEYKLVVVGAVGVGKSALTIEYKLVVVGACGVGKSALTIYKLVVVGAGDVGKSALTIQYKLVVVGAGCVGKSALTIQLLDILDTAGHEEYSAMRDQ

SEQ ID NO: 24 - protein, 119 aa, synthetic construct
YKLVVVGACGVGKSALTYKLVVVGADGVGKSALTYKLVVVGAVGVGKSALTYKLVVVGARGVGKSALTKLVVVGAGCVGKSALTIKLVVVGAGDVGKSALTILDILDTAGHEEYSAMRD

SEQ ID NO: 25 - protein, 167 aa, synthetic construct
LLSVGGYKLVVVGACGVGKSALTLLSVGGYKLVVVGADGVGKSALTLLSVGGYKLVVVGAVGVGKSALTLLSVGGYKLVVVGARGVGKSALTLLSVGGKLVVVGAGCVGKSALTILLSVGGKLVVVGAGDVGKSALTILLSVGGLDILDTAGHEEYSAMRDLLSVGG

SEQ ID NO: 26 - protein, 84 aa, synthetic construct
VGACGVGKSLLSVGGVVVGACGVGLLSVGGVGACGVGKSLLSVGGVVVGACGVGLLSVGGVGACGVGKSLLSVGGVVVGACGVG

SEQ ID NO: 27 - protein, 84 aa, synthetic construct
VGACGVGKSLLSVGGVVVGACGVGLLSVGGVGADGVGKSLLSVGGVVVGADGVGLLSVGGGAGDVGKSALLSVGGVVGAGDVGK

SEQ ID NO: 28 - protein, 147 aa, synthetic construct
MTEYKLVVVGACGVGKSALTIQLIQNHFVDELLSVGGVGACGVGKLLSVGGMTEYKLVVVGADGVGKSALTIQLIQNHFVDELLSVGGVGADGVGKLLSVGGTEYKLVVVGAGDVGKSALTIQLIQNHFVDEYLLSVGGGAGDVGKS

SEQ ID NO: 29 - protein, 216 aa, synthetic construct
MTEYKLVVVGAGCVGKSALTIQLIQNHFVDELLSVGGMTEYKLVVVGACGVGKSALTIQLIQNHFVDELLSVGGMTEYKLVVVGADGVGKSALTIQLIQNHFVDELLSVGGMTEYKLVVVGAGDVGKSALTIQLIQNHFVDELLSVGGMTEYKLVVVGAVGVGKSALTIQLIQNHFVDELLSVGGTCLLDILDTAGHEEYSAMRDQYMRTGEGFLC

SEQ ID NO: 30 - protein, 117 aa, synthetic construct
MTEYKLVVVGACGVGKSALTIQLIQNHFVDEVGACGVGKMTEYKLVVVGADGVGKSALTIQLIQNHFVDEVGADGVGKTEYKLVVVGAGDVGKSALTIQLIQNHFVDEYGAGDVGKS

SEQ ID NO: 31 - protein, 393 aa, synthetic construct
CINLDWDVIRDKTKTKIESLKEHGPIKNKMSESPNKTVSEEKAKQYLEEFHQTALEHPELSELKTVTGTNPVFAGANYAAWAVNVAQVIDSETADNLEKTTAALSILPGIGSVMGIADGAVHHNTEEIVAQSIALSSLMVAQAIPLVGELVDIGFAAYNFVESIINLFQVVHNSYNRMTEYKLVVVGAGCVGKSALTIQLIQNHFVDELLSVGGMTEYKLVVVGACGVGKSALTIQLIQNHFVDELLSVGGMTEYKLVVVGADGVGKSALTIQLIQNHFVDELLSVGGMTEYKLVVVGAGDVGKSALTIQLIQNHFVDELLSVGGMTEYKLVVVGAVGVGKSALTIQLIQNHFVDELLSVGGTCLLDILDTAGHEEYSAMRDQYMRTGEGFLC

SEQ ID NO: 32 - protein, 399 aa, synthetic construct
MTEYKLVVVGAGCVGKSALTIQLIQNHFVDELLSVGGMTEYKLVVVGACGVGKSALTIQLIQNHFVDELLSVGGMTEYKLVVVGADGVGKSALTIQLIQNHFVDELLSVGGMTEYKLVVVGAGDVGKSALTIQLIQNHFVDELLSVGGMTEYKLVVVGAVGVGKSALTIQLIQNHFVDELLSVGGTCLLDILDTAGHEEYSAMRDQYMRTGEGFLCLLSVGGCINLDWDVIRDKTKTKIESLKEHGPIKNKMSESPNKTVSEEKAKQYLEEFHQTALEHPELSELKTVTGTNPVFAGANYAAWAVNVAQVIDSETADNLEKTTAALSILPGIGSVMGIADGAVHHNTEEIVAQSIALSSLMVAQAIPLVGELVDIGFAAYNFVESIINLFQVVHNSYNR

SEQ ID NO: 33 - protein, 399 aa, synthetic construct; identical to SEQ ID NO: 32

SEQ ID NO: 34 - protein, 136 aa, synthetic construct
YKLVVVGACGVGKSALTYKLVVVGADGVGKSALTYKLVVVGAVGVGKSALTYKLVVVGARGVGKSALTKLVVVGAGCVGKSALTIKLVVVGAGDVGKSALTILDILDTAGHEEYSAMRDKLVVVGAGRVGKSALTI

SEQ ID NO: 35 - protein, 402 aa, synthetic construct
MTEYKLVVVGACGVGKSALTIQLIQNHFVDELLSVGGVGACGVGKLLSVGGMTEYKLVVVGADGVGKSALTIQLIQNHFVDELLSVGGVGADGVGKLLSVGGMTEYKLVVVGAVGVGKSALTIQLIQNHFVDELLSVGGVGAVGVGKLLSVGGMTEYKLVVVGARGVGKSALTIQLIQNHFVDELLSVGGVGARGVGKLLSVGGTEYKLVVVGAGCVGKSALTIQLIQNHFVDEYLLSVGGGAGCVGKSLLSVGGTEYKLVVVGAGDVGKSALTIQLIQNHFVDEYLLSVGGGAGDVGKSLLSVGGTCLLDILDTAGHEEYSAMRDQYMRTGEGFLCLLSVGGTAGHEEYSLLSVGGTEYKLVVVGAGRVGKSALTIQLIQNHFVDEYLLSVGGGAGRVGKS

SEQ ID NO: 36 - protein, 312 aa, synthetic construct
MTEYKLVVVGACGVGKSALTIQLIQNHFVDEVGACGVGKMTEYKLVVVGADGVGKSALTIQLIQNHFVDEVGADGVGKMTEYKLVVVGAVGVGKSALTIQLIQNHFVDEVGAVGVGKMTEYKLVVVGARGVGKSALTIQLIQNHFVDEVGARGVGKTEYKLVVVGAGCVGKSALTIQLIQNHFVDEYGAGCVGKSTEYKLVVVGAGDVGKSALTIQLIQNHFVDEYGAGDVGKSTCLLDILDTAGHEEYSAMRDQYMRTGEGFLCTAGHEEYSTEYKLVVVGAGRVGKSALTIQLIQNHFVDEYGAGRVGKS

SEQ ID NO: 37 - protein, 402 aa, synthetic construct
MTEYKLVVVGADGVGKSALTIQLIQNHFVDELLSVGGVGADGVGKLLSVGGMTEYKLVVVGACGVGKSALTIQLIQNHFVDELLSVGGVGACGVGKLLSVGGMTEYKLVVVGAVGVGKSALTIQLIQNHFVDELLSVGGVGAVGVGKLLSVGGMTEYKLVVVGARGVGKSALTIQLIQNHFVDELLSVGGVGARGVGKLLSVGGTEYKLVVVGAGCVGKSALTIQLIQNHFVDEYLLSVGGGAGCVGKSLLSVGGTEYKLVVVGAGDVGKSALTIQLIQNHFVDEYLLSVGGGAGDVGKSLLSVGGTCLLDILDTAGHEEYSAMRDQYMRTGEGFLCLLSVGGTAGHEEYSLLSVGGTEYKLVVVGAGRVGKSALTIQLIQNHFVDEYLLSVGGGAGRVGKS

SEQ ID NO: 38 - protein, 408 aa, synthetic construct
YKLVVVGACGVGKSALTYKLVVVGADGVGKSALTYKLVVVGAVGVGKSALTYKLVVVGARGVGKSALTKLVVVGAGCVGKSALTIKLVVVGAGDVGKSALTILDILDTAGHEEYSAMRDKLVVVGAGRVGKSALTIYKLVVVGACGVGKSALTYKLVVVGADGVGKSALTYKLVVVGAVGVGKSALTYKLVVVGARGVGKSALTKLVVVGAGCVGKSALTILDILDTAGHEEYSAMRDKLVVVGAGDVGKSALTIKLVVVGAGRVGKSALTIYKLVVVGAVGVGKSALTYKLVVVGARGVGKSALTKLVVVGAGCVGKSALTILDILDTAGHEEYSAMRDYKLVVVGACGVGKSALTYKLVVVGADGVGKSALTKLVVVGAGDVGKSALTIKLVVVGAGRVGKSALTI

SEQ ID NO: 39 - protein, 351 aa, synthetic construct
MTEYKLVVVGADGVGKSALTIQLIQNHFVDELLSVGGVGADGVGKLLSVGGMTEYKLVVVGACGVGKSALTIQLIQNHFVDELLSVGGVGACGVGKLLSVGGMTEYKLVVVGAVGVGKSALTIQLIQNHFVDELLSVGGVGAVGVGKLLSVGGMTEYKLVVVGARGVGKSALTIQLIQNHFVDELLSVGGVGARGVGKLLSVGGTEYKLVVVGAGCVGKSALTIQLIQNHFVDEYLLSVGGGAGCVGKSLLSVGGTEYKLVVVGAGDVGKSALTIQLIQNHFVDEYLLSVGGGAGDVGKSLLSVGGTCLLDILDTAGHEEYSAMRDQYMRTGEGFLCLLSVGGTAGHEEYS

SEQ ID NO: 40 - protein, 555 aa, synthetic construct
MTEYKLVVVGADGVGKSALTIQLIQNHFVDELLSVGGVGADGVGKLLSVGGMTEYKLVVVGACGVGKSALTIQLIQNHFVDELLSVGGVGACGVGKLLSVGGMTEYKLVVVGAVGVGKSALTIQLIQNHFVDELLSVGGVGAVGVGKLLSVGGMTEYKLVVVGARGVGKSALTIQLIQNHFVDELLSVGGVGARGVGKLLSVGGTCLLDILDTAGHEEYSAMRDQYMRTGEGFLCLLSVGGTAGHEEYSLLSVGGTEYKLVVVGAGDVGKSALTIQLIQNHFVDEYLLSVGGGAGDVGKSLLSVGGMTEYKLVVVGAAGVGKSALTIQLIQNHFVDELLSVGGVGAAGVGKLLSVGGRSYGIPFIETSTKTRQRVEDAFYTLVREIRQLLSVGGETSTKTRQLLSVGGTEYKLVVVGAGCVGKSALTIQLIQNHFVDEYLLSVGGGAGCVGKSLLSVGGMTEYKLVVVGASGVGKSALTIQLIQNHFVDELLSVGGVGASGVGKLLSVGGTCLLDILDTAGREEYSAMRDQYMRTGEGFLCLLSVGGTAGREEYS

SEQ ID NO: 41 - protein, 402 aa, synthetic construct
MTEYKLVVVGACGVGKSALTIQLIQNHFVDELLSVGGVGACGVGKLLSVGGMTEYKLVVVGAVGVGKSALTIQLIQNHFVDELLSVGGVGAVGVGKLLSVGGMTEYKLVVVGADGVGKSALTIQLIQNHFVDELLSVGGVGADGVGKLLSVGGTCLLDILDTAGHEEYSAMRDQYMRTGEGFLCLLSVGGTAGHEEYSLLSVGGTEYKLVVVGAGCVGKSALTIQLIQNHFVDEYLLSVGGGAGCVGKSLLSVGGTEYKLVVVGAGDVGKSALTIQLIQNHFVDEYLLSVGGGAGDVGKSLLSVGGMTEYKLVVVGAAGVGKSALTIQLIQNHFVDELLSVGGVGAAGVGKLLSVGGMTEYKLVVVGASGVGKSALTIQLIQNHFVDELLSVGGVGASGVGK

SEQ ID NO: 42 - protein, 402 aa, synthetic construct
MTEYKLVVVGADGVGKSALTIQLIQNHFVDELLSVGGVGADGVGKLLSVGGMTEYKLVVVGAVGVGKSALTIQLIQNHFVDELLSVGGVGAVGVGKLLSVGGMTEYKLVVVGARGVGKSALTIQLIQNHFVDELLSVGGVGARGVGKLLSVGGTCLLDILDTAGHEEYSAMRDQYMRTGEGFLCLLSVGGTAGHEEYSLLSVGGTCLLDILDTAGREEYSAMRDQYMRTGEGFLCLLSVGGTAGREEYSLLSVGGTEYKLVVVGAGCVGKSALTIQLIQNHFVDEYLLSVGGGAGCVGKSLLSVGGMTEYKLVVVGACGVGKSALTIQLIQNHFVDELLSVGGVGACGVGKLLSVGGTEYKLVVVGAGDVGKSALTIQLIQNHFVDEYLLSVGGGAGDVGKS

SEQ ID NO: 43 - protein, 402 aa, synthetic construct
MTEYKLVVVGADGVGKSALTIQLIQNHFVDELLSVGGVGADGVGKLLSVGGMTEYKLVVVGAVGVGKSALTIQLIQNHFVDELLSVGGVGAVGVGKLLSVGGTEYKLVVVGAGDVGKSALTIQLIQNHFVDEYLLSVGGGAGDVGKSLLSVGGRSYGIPFIETSTKTRQRVEDAFYTLVREIRQLLSVGGETSTKTRQLLSVGGMTEYKLVVVGACGVGKSALTIQLIQNHFVDELLSVGGVGACGVGKLLSVGGMTEYKLVVVGAAGVGKSALTIQLIQNHFVDELLSVGGVGAAGVGKLLSVGGMTEYKLVVVGASGVGKSALTIQLIQNHFVDELLSVGGVGASGVGKLLSVGGTEYKLVVVGAGCVGKSALTIQLIQNHFVDEYLLSVGGGAGCVGKS

SEQ ID NO: 44 - RNA, 69 nt, synthetic construct
  source 1..69: mol_type = other RNA
atgacagagtacaagctggtggtcgtgggggccaggggcgtgggcaagagcgccctgactatccagctg

SEQ ID NO: 45 - protein, 351 aa, synthetic construct
MTEYKLVMVGADGVGKSALTIQLIQNHFVDELLSVGGVGADGVGKLLSVGGMTEYKLVVVGACGVGKSALTIQLIQNHFVDELLSVGGVGACGVGKLLSVGGMTEYKLVVVGAVGVGKSALTIQLIQNHFVDELLSVGGVGAVGVGKLLSVGGMTEYKLVVVGARGVGKSALTIQLIQNHFVDELLSVGGVGARGVGKLLSVGGTEYKLVVVGAGCVGKSALTIQLIQNHFVDEYLLSVGGGAGCVGKSLLSVGGTEYKLVVVGAGDVGKSALTIQLIQNHFVDEYLLSVGGGAGDVGKSLLSVGGTCLLDILDTAGHEEYSAMRDQYMRTGEGFLCLLSVGGTAGHEEYS

SEQ ID NO: 46 - RNA, 57 nt, synthetic construct
  source 1..57: mol_type = other RNA
gaatacaagctggtggtggtgggcgccgacggcgtggggaagtccgccctcacaatc

SEQ ID NO: 47 - RNA, 57 nt, synthetic construct
  source 1..57: mol_type = other RNA
gagtacaagctggtcgtggtgggggccgtgggcgtcgggaagtccgccctgacaatc

SEQ ID NO: 48 - RNA, 57 nt, synthetic construct
  source 1..57: mol_type = other RNA
gagtacaagttggtggtggtgggcgcctgcggggtgggcaagagcgccctgaccatc

SEQ ID NO: 49 - RNA, 57 nt, synthetic construct
  source 1..57: mol_type = other RNA
tacaagctcgtggtggtgggggccggggacgtggggaagagtgccctgaccatccag

SEQ ID NO: 50 - RNA, 57 nt, synthetic construct
  source 1..57: mol_type = other RNA
tataagctggtggtggtcggcgccgggtgcgtgggcaagtccgccctgacaatccag

SEQ ID NO: 51 - RNA, 57 nt, synthetic construct
  source 1..57: mol_type = other RNA
ctgctggatatcctggataccgccggccacgaggagtacagcgccatgagggatcag

SEQ ID NO: 52 - RNA, 51 nt, synthetic construct
  source 1..51: mol_type = other RNA
tacaagctggtcgtcgtgggggcctgcggcgtggggaagtccgctctgacc

SEQ ID NO: 53 - RNA, 51 nt, synthetic construct
  source 1..51: mol_type = other RNA
tacaaactggtggtggtgggggccgatggggtgggcaagtccgccctgacc

SEQ ID NO: 54 - RNA, 51 nt, synthetic construct
  source 1..51: mol_type = other RNA
tacaagctggtggtggtcggggccgtcggcgtgggcaaaagcgccctgaca

SEQ ID NO: 55 - RNA, 51 nt, synthetic construct
  source 1..51: mol_type = other RNA
tacaagctcgtggtggtgggcgccaggggggtgggcaagtccgccctgaca

SEQ ID NO: 56 - RNA, 51 nt, synthetic construct
  source 1..51: mol_type = other RNA
aagctggtcgtggtgggcgccgggtgcgtgggcaagagcgccctgacaatc

SEQ ID NO: 57 - RNA, 51 nt, synthetic construct
  source 1..51: mol_type = other RNA
aagctggtggtggtgggggccggggatgtgggcaagagcgccctgaccatc

SEQ ID NO: 58 - RNA, 51 nt, synthetic construct
  source 1..51: mol_type = other RNA
ctggacatcctggacacagccgggcacgaggagtacagcgccatgagggat

SEQ ID NO: 59 - RNA, 51 nt, synthetic construct
  source 1..51: mol_type = other RNA
tacaagctcgtggtggtgggcgcctgcggcgtggggaagtccgccctgaca

SEQ ID NO: 60 - RNA, 51 nt, synthetic construct
  source 1..51: mol_type = other RNA
tacaagctggtggtcgtgggcgccgacggggtgggcaagagcgccctcacc

SEQ ID NO: 61 - RNA, 51 nt, synthetic construct
  source 1..51: mol_type = other RNA
tacaagctggtcgtggtcggggccgtgggcgtgggcaagtccgctctgaca

SEQ ID NO: 62 - RNA, 51 nt, synthetic construct
  source 1..51: mol_type = other RNA
tacaagctggtggtggtgggggccaggggggtcgggaaatccgccctgact

SEQ ID NO: 63 - RNA, 51 nt, synthetic construct
  source 1..51: mol_type = other RNA
aagctcgtggtggtgggggccgggtgcgtggggaagtccgccctgacaatt

SEQ ID NO: 64 - RNA, 51 nt, synthetic construct
  source 1..51: mol_type = other RNA
aagctggtcgtggtgggcgccggggatgtgggcaagagcgccctgaccatc

SEQ ID NO: 65 - RNA, 51 nt, synthetic construct
  source 1..51: mol_type = other RNA
ctggacatcctggacaccgccggccacgaggagtacagcgccatgagggat

SEQ ID NO: 66 - RNA, 27 nt, synthetic construct
  source 1..27: mol_type = other RNA
gttggagcctgtggagttggtaaaagt

SEQ ID NO: 67 - RNA, 27 nt, synthetic construct
  source 1..27: mol_type = other RNA
gtagttgtgggagcttgtggagtaggt

SEQ ID NO: 68 - RNA, 27 nt, synthetic construct
  source 1..27: mol_type = other RNA
gtaggagcttgtggagtaggaaagtct

SEQ ID NO: 69 - RNA, 27 nt, synthetic construct
  source 1..27: mol_type = other RNA
gtagtagtaggagcatgcggagtcgga

SEQ ID NO: 70 - RNA, 27 nt, synthetic construct
  source 1..27: mol_type = other RNA
gtaggagcatgcggagtaggaaagtca

SEQ ID NO: 71 - RNA, 27 nt, synthetic construct
  source 1..27: mol_type = other RNA
gtagtagtaggagcttgtggagtagga

SEQ ID NO: 72 - RNA, 27 nt, synthetic construct
  source 1..27: mol_type = other RNA
gtgggcgcctgtggagtaggaaaatct

SEQ ID NO: 73 - RNA, 27 nt, synthetic construct
  source 1..27: mol_type = other RNA
gtggtggtcggagcatgcggagtagga

SEQ ID NO: 74 - RNA, 27 nt, synthetic construct
  source 1..27: mol_type = other RNA
gtgggagctgacggcgtgggtaaatcc

SEQ ID NO: 75 - RNA, 27 nt, synthetic construct
  source 1..27: mol_type = other RNA
gtggtcgtgggagctgacggtgttggt

SEQ ID NO: 76 - RNA, 27 nt, synthetic construct
  source 1..27: mol_type = other RNA
ggagcgggagatgttggaaagtcagcc

SEQ ID NO: 77 - RNA, 27 nt, synthetic construct
  source 1..27: mol_type = other RNA
gttgtgggggctggtgacgtgggaaag

SEQ ID NO: 78 - RNA, 93 nt, synthetic construct
  source 1..93: mol_type = other RNA
atgacagaatacaaacttgtggtagttggagcatgcggtgtgggtaagagtgccctcaccatccaactaattcagaaccacttcgttgacgaa

SEQ ID NO: 79 - RNA, 24 nt, synthetic construct
  source 1..24: mol_type = other RNA
gttggagcatgtggtgtagggaag

SEQ ID NO: 80 - RNA, 93 nt, synthetic construct
  source 1..93: mol_type = other RNA
atgactgaatacaaacttgtggttgttggagcagatggggtcggaaaatccgccttgacaatacagcttattcagaatcactttgtggatgag

SEQ ID NO: 81 - RNA, 24 nt, synthetic construct
  source 1..24: mol_type = other RNA
gtcggagctgatggcgtcggaaag

SEQ ID NO: 82 - RNA, 93 nt, synthetic construct
  source 1..93: mol_type = other RNA
actgagtataaattagtggtagtcggggctggagacgtgggcaagagtgcccttaccatccagctcatccagaatcattttgtggacgagtat

SEQ ID NO: 83 - RNA, 24 nt, synthetic construct
  source 1..24: mol_type = other RNA
ggagctggtgacgtcggaaagtct

SEQ ID NO: 84 - RNA, 93 nt, synthetic construct
  source 1..93: mol_type = other RNA
atgactgaatataaactcgtcgtggttggagcaggttgcgttggcaaaagcgcccttacaatccagctgatacagaaccacttcgtggatgag

SEQ ID NO: 85 - RNA, 93 nt, synthetic construct
  source 1..93: mol_type = other RNA
atgacagagtacaagttggtggtggtgggcgcctgtggggtggggaaatctgcccttactatccagctgatccagaaccactttgtggatgag

SEQ ID NO: 86 - RNA, 93 nt, synthetic construct
  source 1..93: mol_type = other RNA
atgacagaatacaaactggtcgtggtcggcgctgatggcgttgggaagagtgctctgacaattcaactcatccagaatcacttcgtagacgaa

SEQ ID NO: 87 - RNA, 93 nt, synthetic construct
  source 1..93: mol_type = other RNA
atgacggagtataagctcgttgtggtaggcgccggagacgtaggcaagtccgcactgaccattcagctcattcaaaatcattttgtagacgaa

SEQ ID NO: 88 - RNA, 93 nt, synthetic construct
  source 1..93: mol_type = other RNA
atgaccgagtacaagctggttgttgtgggtgccgtgggggtgggtaagtcagccctcaccattcagctcatccaaaaccatttcgtggacgag

SEQ ID NO: 89 - RNA, 93 nt, synthetic construct
  source 1..93: mol_type = other RNA
acctgcctcctggacatattggacactgcggggcatgaggagtattccgcaatgcgcgatcagtacatgaggaccggagaaggatttctgtgc

SEQ ID NO: 90 - RNA, 93 nt, synthetic construct
  source 1..93: mol_type = other RNA
atgacagagtataagctggtcgtggtcggcgcgtgcggagtggggaaatcagctctcaccattcagctaatccagaaccacttcgttgacgaa

SEQ ID NO: 91 - RNA, 24 nt, synthetic construct
  source 1..24: mol_type = other RNA
gtcggcgcttgcggtgtcggaaag

SEQ ID NO: 92 - RNA, 93 nt, synthetic construct
  source 1..93: mol_type = other RNA
atgacggagtataaacttgtcgtagttggcgccgacggtgttggaaaatccgcattaaccatacaattgatccagaaccacttcgtggacgaa

SEQ ID NO: 93 - RNA, 24 nt, synthetic construct
  source 1..24: mol_type = other RNA
gtgggggctgacggcgtaggaaaa

SEQ ID NO: 94 - RNA, 93 nt, synthetic construct
  source 1..93: mol_type = other RNA
acagagtacaagctggtggtggttggcgcaggggatgtgggtaagagcgccctgactattcagctgatccaaaatcattttgtggatgaatac

SEQ ID NO: 95 - RNA, 24 nt, synthetic construct
  source 1..24: mol_type = other RNA
ggagcaggcgatgtggggaagtct

SEQ ID NO: 96 - RNA, 531 nt, synthetic construct
  source 1..531: mol_type = other RNA
tgtataaacctcgattgggatgtaatccgcgacaaaaccaagacaaaaattgaatctctcaaggagcacggccctatcaaaaataaaatgtcagagtcacccaataagacggtgtctgaggaaaaggccaagcaatacttggaagaatttcatcaaaccgccttggaacatccggaactaagcgagcttaagacagttacaggtactaacccagtgtttgccggagctaactacgccgcgtgggcggtcaatgtagcccaggtcattgatagtgaaactgctgacaatttagaaaagacaactgccgctctctccattctgcccggaatagggagcgttatgggtatcgcagatggcgcggtgcatcataacaccgaggagatcgtcgcacagtcgatcgctctcagtagcctaatggtggctcaggcaattcctctggtcggggaactggttgacatcggattcgccgcatacaatttcgtagagtctattataaatcttttccaggtggtccacaactcatataatcga

SEQ ID NO: 97 - RNA, 93 nt, synthetic construct
  source 1..93: mol_type = other RNA
atgactgagtacaagctggtagtggtaggggctggatgcgtcgggaagtcagccctgactatacagctgatccagaaccacttcgtggatgag

SEQ ID NO: 98 - RNA, 93 nt, synthetic construct
  source 1..93: mol_type = other RNA
atgacggaatataagctcgttgtggtaggggcttgtggagtgggcaagtccgcactgacaatccagctgatccagaatcactttgtggatgag

SEQ ID NO: 99 - RNA, 93 nt, synthetic construct
  source 1..93: mol_type = other RNA
atgaccgaatacaaacttgttgtggtgggcgctgacggagttggtaaaagcgcccttaccatccaactgattcagaaccactttgtcgacgag

SEQ ID NO: 100 - RNA, 93 nt, synthetic construct
  source 1..93: mol_type = other RNA
atgaccgagtataaattggtggtggtgggcgctggcgacgtgggcaaaagtgcactgacaattcagctgattcagaaccactttgtggacgag

SEQ ID NO: 101 - RNA, 93 nt, synthetic construct
  source 1..93: mol_type = other RNA
atgaccgagtataagttggtggttgtcggcgcggttggtgtgggaaaatctgcccttacaatccagctgattcaaaaccatttcgtcgacgag

SEQ ID NO: 102 - RNA, 93 nt, synthetic construct
  source 1..93: mol_type = other RNA
acgtgcttgctcgacatcctggatactgccggccacgaagagtactccgccatgcgggatcaatatatgcgtaccggcgaggggttcttatgt

SEQ ID NO: 103 - RNA, 93 nt, synthetic construct
  source 1..93: mol_type = other RNA
atgacagagtacaagctggtggtcgtcggagccggttgcgtaggaaagagcgcattaaccatccagctaatccaaaaccatttcgtggacgaa

SEQ ID NO: 104 - RNA, 93 nt, synthetic construct
  source 1..93: mol_type = other RNA
atgactgaatacaagttagtggtggttggggcctgtggtgtgggaaaatccgctctcacgatccagctgattcagaaccacttcgtcgacgag

SEQ ID NO: 105 - RNA, 93 nt, synthetic construct
  source 1..93: mol_type = other RNA
atgaccgaatataaactggttgtcgtgggggctgatggagttggcaagtctgccttgactattcaactgatccagaatcattttgtggatgag

SEQ ID NO: 106 - RNA, 93 nt, synthetic construct
  source 1..93: mol_type = other RNA
atgacagagtataaactcgtcgtggtgggtgccggagatgttgggaaatctgctcttaccatacagttaatccaaaatcacttcgttgatgaa

SEQ ID NO: 107 - RNA, 93 nt, synthetic construct
  source 1..93: mol_type = other RNA
atgactgagtacaagttggtggtggtgggggctgtgggggtgggaaagtctgcactgactattcagctcattcagaaccacttcgtggatgag

SEQ ID NO: 108 - RNA, 93 nt, synthetic construct
  source 1..93: mol_type = other RNA
acctgtctgctagacattctggacacggccggccatgaggagtatagcgcaatgagagaccaatacatgcggaccggcgaaggctttctttgc

SEQ ID NO: 109 - RNA, 531 nt, synthetic construct
  source 1..531: mol_type = other RNA
tgtataaacctcgactgggatgtgatccgcgataaaaccaagaccaagatcgaaagcctaaaggagcatggccctattaagaataaaatgtcagaatctcccaataaaacagtatccgaggaaaaggccaaacagtatttggaagagtttcaccagaccgccctggaacacccagagctgtccgaactgaagacagtcactgggacaaatcctgtcttcgccggtgctaactacgcggcatgggcggtcaatgtagcccaagttatcgatagtgagactgccgacaaccttgagaaaaccacagcagcattgagcatattgccgggcatcggttctgtcatgggcatagctgacggcgctgtgcaccacaacacagaggagatcgtcgctcagagtattgcgctgtccagtcttatggtggcccaggccatcccacttgttggtgaactggtggacatcggatttgcagcgtacaactttgtcgagtcaattattaatctgttccaggttgtccataacagttataatcgt

SEQ ID NO: 110 - RNA, 261 nt, synthetic construct
  source 1..261: mol_type = other RNA
tgtataaatcttgactgggacgtcattagggataagacaaagaccaagatagagtccttgaaggagcacggccccatcaaaaacaaaatgtcggagagcccaaacaaaacagtgagtgaagagaaagcaaagcagtatcttgaagagtttcaccagacggctctggaacatcctgagctgtctgaacttaagacagtgaccggcacaaaccctgtgtttgcaggagctaattatgcggcttgggccgttaacgtggctcag

SEQ ID NO: 111 - RNA, 93 nt, synthetic construct
  source 1..93: mol_type = other RNA
atgactgagtataaactggttgtggtgggcgccggctgcgtcggaaagagcgcgctgaccattcaacttattcaaaatcacttcgttgatgaa

SEQ ID NO: 112 - RNA, 93 nt, synthetic construct
  source 1..93: mol_type = other RNA
atgactgaatataagttagtggtcgtgggcgcctgtggggtgggtaaaagcgccctaactatacagctaatccagaaccactttgtagacgag

SEQ ID NO: 113 - RNA, 93 nt, synthetic construct
  source 1..93: mol_type = other RNA
atgacagagtacaagctggtggttgtaggtgcagacggcgtcggcaaatccgccctcactatccagctgattcagaaccactttgtagacgag

SEQ ID NO: 114 - RNA, 93 nt, synthetic construct
  source 1..93: mol_type = other RNA
atgactgaatacaaacttgttgtggttggggctggggatgtcggaaagagtgctctgacgattcagctgatccagaaccattttgtggacgaa

SEQ ID NO: 115 - RNA, 93 nt, synthetic construct
  source 1..93: mol_type = other RNA
atgaccgagtacaagctggtggttgtgggagcggtcggggtcgggaagtccgccttaacaatccagctgatccaaaatcacttcgtggatgaa

SEQ ID NO: 116 - RNA, 93 nt, synthetic construct
  source 1..93: mol_type = other RNA
acctgcctgctcgacatcctcgataccgccggtcacgaagagtactccgccatgcgtgatcaatatatgcgaacgggggagggtttcttatgc

SEQ ID NO: 117 - RNA, 246 nt, synthetic construct
  source 1..246: mol_type = other RNA
aatttggagaaaaccaccgcagcactatctatcctgccgggaataggtagcgtcatgggcatcgccgacggagcagtacatcataatactgaagaaattgtggcccaatctatcgccttaagttctttgatggtggctcaggctattcccctggtcggggagctggtagatattggcttcgctgcctacaacttcgtggagagcatcattaatttgttccaggtcgtgcataatagctacaacagg

SEQ ID NO: 118 - RNA, 51 nt, synthetic construct
  source 1..51: mol_type = other RNA
tacaagctagtggtggtcggcgcatgcggcgtgggaaagagcgcgctaacc

SEQ ID NO: 119 - RNA, 51 nt, synthetic construct
  source 1..51: mol_type = other RNA
tataaattggtcgttgtgggcgccgatggtgtagggaaatctgcgctgacc

SEQ ID NO: 120 - RNA, 51 nt, synthetic construct
  source 1..51: mol_type = other RNA
tacaagctcgtggtggtgggggcagtcggcgtcggcaaaagtgccctgact

SEQ ID NO: 121 - RNA, 51 nt, synthetic construct
  source 1..51: mol_type = other RNA
tataagctggtcgtggtaggtgctcgtggcgttggaaagtccgccttgaca

SEQ ID NO: 122 - RNA, 51 nt, synthetic construct
  source 1..51: mol_type = other RNA
aagctggttgtcgtgggggccggatgcgtgggcaaatctgctcttacaatc

SEQ ID NO: 123 - RNA, 51 nt, synthetic construct
  source 1..51: mol_type = other RNA
aaattagtagttgtgggagctggagacgtaggtaaatccgcactgacgata

SEQ ID NO: 124 - RNA, 51 nt, synthetic construct
  source 1..51: mol_type = other RNA
ctcgatattctcgacaccgctggacacgaagagtacagcgccatgcgcgac

SEQ ID NO: 125 - RNA, 51 nt, synthetic construct
  source 1..51: mol_type = other RNA
aagctggtcgtggtgggggccggcagagttggtaagtcagcactcactatc

SEQ ID NO: 126 - RNA, 93 nt, synthetic construct
  source 1..93: mol_type = other RNA
atgaccgagtacaaactcgttgtggtgggggcctgcggagtgggcaagtctgcattgaccatacagttgatccagaatcatttcgtggatgag

SEQ ID NO: 127 - RNA, 24 nt, synthetic construct
  source 1..24: mol_type = other RNA
gtcggagcgtgtggcgtgggcaaa

SEQ ID NO: 128 - RNA, 93 nt, synthetic construct
  source 1..93: mol_type = other RNA
atgactgagtataagttagtagtcgttggtgccgatggagtaggcaaatcggcgttaacgatccagcttattcagaatcatttcgtagatgag

SEQ ID NO: 129 - RNA, 24 nt, synthetic construct
  source 1..24: mol_type = other RNA
gtcggggccgacggcgtgggcaaa

SEQ ID NO: 130 - RNA, 93 nt, synthetic construct
  source 1..93: mol_type = other RNA
atgaccgagtataagttagtcgtcgtgggtgctgtgggcgtaggtaaatccgccctgactatacagcttattcaaaaccattttgtggatgag

SEQ ID NO: 131 - RNA, 24 nt, synthetic construct
  source 1..24: mol_type = other RNA
gtgggagctgtgggcgttgggaaa

SEQ ID NO: 132 - RNA, 93 nt, synthetic construct
  source 1..93: mol_type = other RNA
atgactgagtacaagctggtggtcgtcggtgcccggggcgttggtaagagcgccctgaccatacaactcattcagaaccactttgtagacgaa

SEQ ID NO: 133 - RNA, 24 nt, synthetic construct
  source 1..24: mol_type = other RNA
gtgggagcaaggggagtcgggaaa

SEQ ID NO: 134 - RNA, 93 nt, synthetic construct
  source 1..93: mol_type = other RNA
acagaatacaagctggttgtagtcggcgccggttgtgtcgggaagtccgcactcacaattcagcttatccagaatcacttcgtggacgagtat

SEQ ID NO: 135 - RNA, 24 nt, synthetic construct
  source 1..24: mol_type = other RNA
ggggcaggctgcgttggaaagagc

SEQ ID NO: 136 - RNA, 93 nt, synthetic construct
  source 1..93: mol_type = other RNA
acagagtacaaattagtggtcgtgggagctggggacgtgggaaagtccgctctcactatccagctgattcagaaccattttgtcgacgaatat

SEQ ID NO: 137 - RNA, 24 nt, synthetic construct
  source 1..24: mol_type = other RNA
ggggctggggacgtgggcaaatca

SEQ ID NO: 138 - RNA, 93 nt, synthetic construct
  source 1..93: mol_type = other RNA
acctgcctgctggatatcctggacacagcgggacacgaagaatacagcgccatgagagatcagtacatgcgaacgggtgaaggcttcctgtgc

SEQ ID NO: 139 - RNA, 24 nt, synthetic construct
  source 1..24: mol_type = other RNA
acagcagggcacgaggaatactcc

SEQ ID NO: 140 - RNA, 93 nt, synthetic construct
  source 1..93: mol_type = other RNA
actgaatataagctggtagttgttggcgcaggaagagttgggaagagtgctctaaccatccaacttatccagaaccactttgtggacgagtat

SEQ ID NO: 141 - RNA, 24 nt, synthetic construct
  source 1..24: mol_type = other RNA
ggcgccgggcgcgtcggaaagtct

SEQ ID NO: 142 - RNA, 93 nt, synthetic construct
  source 1..93: mol_type = other RNA
atgacagaatacaagttagtggtggtaggagcgtgtggagtggggaaaagcgccctaactattcagttgatacaaaaccatttcgtggacgaa

SEQ ID NO: 143 - RNA, 24 nt, synthetic construct
  source 1..24: mol_type = other RNA
gtgggcgcatgtggagtcggcaag

SEQ ID NO: 144 - RNA, 93 nt, synthetic construct
  source 1..93: mol_type = other RNA
atgaccgagtataagctcgtagtcgtgggggccgacggcgtggggaaatcagcccttactatccagcttatacaaaaccattttgttgacgaa

SEQ ID NO: 145 - RNA, 24 nt, synthetic construct
  source 1..24: mol_type = other RNA
gtaggcgccgacggggtcggaaag

SEQ ID NO: 146 - RNA, 93 nt, synthetic construct
  source 1..93: mol_type = other RNA
atgaccgagtacaagctggttgtcgtcggggccgtaggggttggcaaaagcgccctgactatccagctcatccaaaatcatttcgtcgacgag

SEQ ID NO: 147 - RNA, 24 nt, synthetic construct
  source 1..24: mol_type = other RNA
gtgggcgccgttggagtcggtaaa

SEQ ID NO: 148 - RNA, 93 nt, synthetic construct
  source 1..93: mol_type = other RNA
atgacggaatacaagttggtggtagtgggggctcggggggtgggcaagagtgctttgaccatacagttaattcagaaccactttgtggatgag

SEQ ID NO: 149 - RNA, 24 nt, synthetic construct
  source 1..24: mol_type = other RNA
gtcggcgctcgcggagtcggcaaa

SEQ ID NO: 150 - RNA, 93 nt, synthetic construct
  source 1..93: mol_type = other RNA
accgagtataaattggttgttgtcggcgcaggctgtgtgggcaagtctgctctcaccattcaactaatccagaaccactttgttgatgagtac

SEQ ID NO: 151 - RNA, 24 nt, synthetic construct
  source 1..24: mol_type = other RNA
ggagcaggctgcgtgggaaaaagc

SEQ ID NO: 152 - RNA, 93 nt, synthetic construct
  source 1..93: mol_type = other RNA
acggagtacaagctggttgtcgtaggagcaggagacgtgggcaaatccgctctgacaattcagcttatccagaatcactttgtggatgaatat

SEQ ID NO: 153 - RNA, 24 nt, synthetic construct
  source 1..24: mol_type = other RNA
ggtgccggggatgtcggtaaaagt

SEQ ID NO: 154 - RNA, 93 nt, synthetic construct
  source 1..93: mol_type = other RNA
acctgcttactggacatcctggacactgctggtcacgaggaatactccgcgatgcgagatcagtatatgcggacaggagagggtttcctgtgc

SEQ ID NO: 155 - RNA, 24 nt, synthetic construct
  source 1..24: mol_type = other RNA
acagcaggccatgaggaatattct

SEQ ID NO: 156 - RNA, 93 nt, synthetic construct
  source 1..93: mol_type = other RNA
actgaatataagctggtggtggtgggggctggtagagtggggaagtcagcactgacaatccagctcattcagaatcacttcgttgatgagtac

SEQ ID NO: 157 - RNA, 24 nt, synthetic construct
  source 1..24: mol_type = other RNA
ggtgcgggtagagtgggcaagtcc

SEQ ID NO: 158 - RNA, 93 nt, synthetic construct
  source 1..93: mol_type = other RNA
atgacggaatacaagctcgtcgtggtgggcgccgatggcgtcggcaagtcggcactgactatccagctcatacaaaatcattttgttgatgaa

SEQ ID NO: 159 - RNA, 24 nt, synthetic construct
  source 1..24: mol_type = other RNA
gtgggggcggacggagtggggaag

SEQ ID NO: 160 - RNA, 93 nt, synthetic construct
  source 1..93: mol_type = other RNA
atgaccgaatacaaactggtggtggtcggggcgtgtggggtgggcaaatcagccctcacaatacagctgattcagaaccactttgttgacgag

SEQ ID NO: 161 - RNA, 24 nt, synthetic construct
  source 1..24: mol_type = other RNA
gtgggggcatgtggagtggggaag

SEQ ID NO: 162 - RNA, 93 nt, synthetic construct
  source 1..93: mol_type = other RNA
atgactgagtacaagctggttgttgtaggtgctgttggagtgggaaagagcgccctcacaatccaattgatccagaatcacttcgtcgacgag

SEQ ID NO: 163 - RNA, 24 nt, synthetic construct
  source 1..24: mol_type = other RNA
gtgggggccgtaggcgtgggcaag

SEQ ID NO: 164 - RNA, 93 nt, synthetic construct
  source 1..93: mol_type = other RNA
atgaccgaatataagttggtagtggtgggggctcgcggagtcgggaagagtgctcttactattcagctgattcagaaccatttcgtagatgaa

SEQ ID NO: 165 - RNA, 24 nt, synthetic construct
  source 1..24: mol_type = other RNA
gtgggcgccagaggcgtgggcaaa

SEQ ID NO: 166 - RNA, 93 nt, synthetic construct
  source 1..93: mol_type = other RNA
actgagtacaaactagtagtcgtaggagctgggtgtgtgggcaaaagtgcactcaccatccagctgatccagaaccatttcgtggatgagtat

SEQ ID NO: 167 - RNA, 24 nt, synthetic construct
  source 1..24: mol_type = other RNA
ggagctggctgcgtgggcaaaagc

SEQ ID NO: 168 - RNA, 93 nt, synthetic construct
  source 1..93: mol_type = other RNA
acggaatacaaactagttgttgtgggggctggtgatgtcggaaagtccgccttgactattcagcttattcaaaatcactttgtcgacgagtat

SEQ ID NO: 169 - RNA, 24 nt, synthetic construct
  source 1..24: mol_type = other RNA
ggcgcaggtgacgtaggaaagtct

SEQ ID NO: 170 - RNA, 93 nt, synthetic construct
  source 1..93: mol_type = other RNA
acctgccttctggacatcctggacacagccggccacgaggaatacagcgccatgcgggatcagtatatgaggacaggagaaggcttcctctgc

SEQ ID NO: 171 - RNA, 24 nt, synthetic construct
  source 1..24: mol_type = other RNA
acagctggccacgaggagtattct

SEQ ID NO: 172 - RNA, 93 nt, synthetic construct
  source 1..93: mol_type = other RNA
accgagtacaaacttgtggtggttggagcagggcgtgtcggcaaatctgccctgaccatccagctgatacaaaaccattttgtggatgagtat

SEQ ID NO: 173 - RNA, 27 nt, synthetic construct
  source 1..27: mol_type = other RNA
ggcggtgcgggacgagtgggcaagagc

SEQ ID NO: 174 - RNA, 51 nt, synthetic construct
  source 1..51: mol_type = other RNA
tataagttggtggtggttggggcatgtggcgtaggtaagagcgcactgact

SEQ ID NO: 175 - RNA, 51 nt, synthetic construct
  source 1..51: mol_type = other RNA
tataagctagttgtcgtgggagctgacggagtggggaagagtgcactcaca

SEQ ID NO: 176 - RNA, 51 nt, synthetic construct
  source 1..51: mol_type = other RNA
tacaagctcgtcgtggtgggcgccgtcggcgtagggaaatcagctcttacc

SEQ ID NO: 177 - RNA, 51 nt, synthetic construct
  source 1..51: mol_type = other RNA
tataaactcgtggtggtgggcgctcgcggtgtgggcaaaagtgccctgacc

SEQ ID NO: 178 - RNA, 51 nt, synthetic construct
  source 1..51: mol_type = other RNA
aagctggtcgtcgtgggcgccggctgcgttgggaaatccgccctgacaatc

SEQ ID NO: 179 - RNA, 51 nt, synthetic construct
  source 1..51: mol_type = other RNA
aaattggtcgtcgtgggcgccggggacgtgggtaagtcagccttgaccatc

SEQ ID NO: 180 - RNA, 51 nt, synthetic construct
  source 1..51: mol_type = other RNA
aaattagtggtggtaggtgccggtagagtggggaagtcggctctcaccatt

SEQ ID NO: 181 - RNA, 51 nt, synthetic construct
  source 1..51: mol_type = other RNA
ctcgacatactggacactgccggccacgaagaatattctgccatgagggat

SEQ ID NO: 182 - RNA, 51 nt, synthetic construct
  source 1..51: mol_type = other RNA
tacaagctggtggtagtcggcgcatgtggagtgggaaaaagcgccctgaca

SEQ ID NO: 183 - RNA, 51 nt, synthetic construct
  source 1..51: mol_type = other RNA
tacaaattagtggtggtcggtgctgatggggtcggcaagtcagctctgacc

SEQ ID NO: 184 - RNA, 51 nt, synthetic construct
  source 1..51: mol_type = other RNA
tacaaactcgttgtcgttggggccgtcggagtgggtaaatccgccctgacc

SEQ ID NO: 185 - RNA, 51 nt, synthetic construct
  source 1..51: mol_type = other RNA
tataaattggtcgtggtaggggctcggggagtcgggaaatctgcgctgacc

SEQ ID NO: 186 - RNA, 51 nt, synthetic construct
  source 1..51: mol_type = other RNA
aagctcgttgtggtgggagcaggttgcgttggtaagtctgctttgactatc

SEQ ID NO: 187 - RNA, 51 nt, synthetic construct
  source 1..51: mol_type = other RNA
ctcgacatcctcgacaccgcaggacatgaggagtactccgccatgcgtgac

SEQ ID NO: 188 - RNA, 51 nt, synthetic construct
  source 1..51: mol_type = other RNA
aagctagtagttgtaggagccggtgatgtgggaaagtccgctctgacaatt

SEQ ID NO: 189 - RNA, 51 nt, synthetic construct
  source 1..51: mol_type = other RNA
aaattggtagtcgtgggggccggcagagtgggaaaaagcgcgctgacaatc

SEQ ID NO: 190 - RNA, 51 nt, synthetic construct
  source 1..51: mol_type = other RNA
tataaacttgttgtggtgggcgcagtcggagttggtaagtcagctctgact

SEQ ID NO: 191 - RNA, 51 nt, synthetic construct
  source 1..51: mol_type = other RNA
tacaagctcgttgttgtgggcgctcgcggggtgggcaagtctgccctaaca

SEQ ID NO: 192 - RNA, 51 nt, synthetic construct
  source 1..51: mol_type = other RNA
aaactagtggtggtcggcgccgggtgcgtaggaaagagtgctctgaccata

SEQ ID NO: 193 - RNA, 51 nt, synthetic construct
  source 1..51: mol_type = other RNA
cttgacattctggatactgcgggccacgaggaatatagcgcgatgcgagat

SEQ ID NO: 194 - RNA, 51 nt, synthetic construct
  source 1..51: mol_type = other RNA
tacaaactggttgttgtgggagcatgtggcgtcgggaagtccgcattaacg

SEQ ID NO: 195 - RNA, 51 nt, synthetic construct
  source 1..51: mol_type = other RNA
tacaagttagtggtggtcggagcggatggcgttgggaagtctgcacttacg

SEQ ID NO: 196 - RNA, 51 nt, synthetic construct
  source 1..51: mol_type = other RNA
aagttggtggtggtgggggccggagacgtaggcaagtccgcacttaccatc

SEQ ID NO: 197 - RNA, 51 nt, synthetic construct
  source 1..51: mol_type = other RNA
aaactggttgtcgtcggcgccgggcgggtgggcaagagcgcactgactatt

SEQ ID NO: 198 - RNA, 93 nt, synthetic construct; identical to SEQ ID NO: 158
  source 1..93: mol_type = other RNA

SEQ ID NO: 199 - RNA, 24 nt, synthetic construct
  source 1..24: mol_type = other RNA
gtgggggcggacggagtggggaag

SEQ ID NO: 200 - RNA, 93 nt, synthetic construct; identical to SEQ ID NO: 160
  source 1..93: mol_type = other RNA

SEQ ID NO: 201 - RNA, 24 nt, synthetic construct
  source 1..24: mol_type = other RNA
gtgggggcatgtggagtggggaag

SEQ ID NO: 202 - RNA, 93 nt, synthetic construct; identical to SEQ ID NO: 162
  source 1..93: mol_type = other RNA

SEQ ID NO: 203 - RNA, 24 nt, synthetic construct
  source 1..24: mol_type = other RNA
gtgggggccgtaggcgtgggcaag

SEQ ID NO: 204 - RNA, 93 nt, synthetic construct; identical to SEQ ID NO: 164
  source 1..93: mol_type = other RNA

SEQ ID NO: 205 - RNA, 24 nt, synthetic construct
  source 1..24: mol_type = other RNA
gtgggcgccagaggcgtgggcaaa

SEQ ID NO: 206 - RNA, 93 nt, synthetic construct; identical to SEQ ID NO: 166
  source 1..93: mol_type = other RNA

SEQ ID NO: 207 - RNA, 24 nt, synthetic construct
  source 1..24: mol_type = other RNA
ggagctggctgcgtgggcaaaagc

SEQ ID NO: 208 - RNA, 93 nt, synthetic construct; identical to SEQ ID NO: 168
  source 1..93: mol_type = other RNA

SEQ ID NO: 209 - RNA, 24 nt, synthetic construct
  source 1..24: mol_type = other RNA
ggcgcaggtgacgtaggaaagtct

SEQ ID NO: 210 - RNA, 93 nt, synthetic construct; identical to SEQ ID NO: 170
  source 1..93: mol_type = other RNA

SEQ ID NO: 211 - RNA, 24 nt, synthetic construct
  source 1..24: mol_type = other RNA
acagctggccacgaggagtattct

SEQ ID NO: 212 - RNA, 93 nt, synthetic construct
  source 1..93: mol_type = other RNA
atgacagagtataaactcgtggtggtcggcgcagatggcgttggaaagagcgccctgactattcagctcatccagaaccatttcgtagacgaa

SEQ ID NO: 213 - RNA, 24 nt, synthetic construct
  source 1..24: mol_type = other RNA
gtcggcgcagacggtgtgggaaag

SEQ ID NO: 214 - RNA, 93 nt, synthetic construct
  source 1..93: mol_type = other RNA
atgaccgaatacaagttagtggtggtcggggcctgcggtgtgggtaaaagcgctctgaccatacagcttatccagaaccacttcgtggatgag

SEQ ID NO: 215 - RNA, 24 nt, synthetic construct
  source 1..24: mol_type = other RNA
gtgggggcttgcggagttggcaag

SEQ ID NO: 216 - RNA, 93 nt, synthetic construct
  source 1..93: mol_type = other RNA
atgacagaatataaattggtggtagtgggggccgtaggcgtcggcaagagcgccctgactatacaactgatccaaaaccacttcgtggacgag

SEQ ID NO: 217 - RNA, 24 nt, synthetic construct
  source 1..24: mol_type = other RNA
gtgggcgccgttggagtcgggaaa

SEQ ID NO: 218 - RNA, 93 nt, synthetic construct
  source 1..93: mol_type = other RNA
atgactgagtataaacttgttgtagtcggggcacggggcgtgggaaagtccgctttaaccatacaattgatacagaaccactttgttgatgaa

SEQ ID NO: 219 - RNA, 24 nt, synthetic construct
  source 1..24: mol_type = other RNA
gtgggtgccaggggagtcggtaag

SEQ ID NO: 220 - RNA, 93 nt, synthetic construct
  source 1..93: mol_type = other RNA
acctgtctcctagacattctggacacagccggccacgaggagtactcagctatgcgcgatcagtatatgagaacaggggagggatttctgtgt

SEQ ID NO: 221 - RNA, 24 nt, synthetic construct
  source 1..24: mol_type = other RNA
acagcagggcacgaagagtacagc

SEQ ID NO: 222 - RNA, 93 nt, synthetic construct
  source 1..93: mol_type = other RNA
actgagtacaagctagtcgtggttggcgcaggcgacgtgggtaaatctgccctcaccattcagttaattcagaatcatttcgtcgatgaatat

SEQ ID NO: 223 - RNA, 24 nt, synthetic construct
  source 1..24: mol_type = other RNA
ggcgctggagacgtcggcaaatcc

SEQ ID NO: 224 - RNA, 93 nt, synthetic construct
  source 1..93: mol_type = other RNA
atgacggagtataaactggtagtcgtaggtgctgccggcgtcggcaaaagcgcgctaaccatccagctgatccagaatcactttgtggatgaa

SEQ ID NO: 225 - RNA, 24 nt, synthetic construct
  source 1..24: mol_type = other RNA
gtgggagccgctggagtggggaag

SEQ ID NO: 226 - RNA, 93 nt, synthetic construct
  source 1..93: mol_type = other RNA
agatcttacggaatccctttcatcgaaacctcaaccaagactcgtcaaagggttgaagacgctttctatacacttgtcagagagattaggcag

SEQ ID NO: 227 - RNA, 24 nt, synthetic construct
  source 1..24: mol_type = other RNA
gaaacctccacaaagacgcggcaa

SEQ ID NO: 228 - RNA, 93 nt, synthetic construct
  source 1..93: mol_type = other RNA
actgagtacaagctggtggtagtgggagccggttgcgtgggcaagtcagcgctgacaatccagctcatccagaatcattttgttgatgagtac

SEQ ID NO: 229 - RNA, 24 nt, synthetic construct
  source 1..24: mol_type = other RNA
ggcgcaggctgcgtggggaaatcg

SEQ ID NO: 230 - RNA, 93 nt, synthetic construct
  source 1..93: mol_type = other RNA
atgactgagtacaagctggtggtggtgggggcgtctggggtggggaaatctgcactgacgattcaactgatccagaatcattttgtagacgag

SEQ ID NO: 231 - RNA, 24 nt, synthetic construct
  source 1..24: mol_type = other RNA
gtgggcgcgtccggcgtgggtaag

SEQ ID NO: 232 - RNA, 93 nt, synthetic construct
  source 1..93: mol_type = other RNA
acctgtttgctggatattctggacactgccggacgagaagaatacagtgcaatgagggatcagtatatgcgaaccggagagggctttctttgt

SEQ ID NO: 233 - RNA, 24 nt, synthetic construct
  source 1..24: mol_type = other RNA
acagccggccgcgaagagtacagc

SEQ ID NO: 234 - RNA, 93 nt, synthetic construct
  source 1..93: mol_type = other RNA
atgacggaatataagctcgtggtcgttggggcctgtggcgtgggtaagagcgcactaaccattcagttaatccagaaccactttgttgatgaa

SEQ ID NO: 235 - RNA, 24 nt, synthetic construct
  source 1..24: mol_type = other RNA
gttggggcctgcggcgttggaaaa

SEQ ID NO: 236 - RNA, 93 nt, synthetic construct
  source 1..93: mol_type = other RNA
atgacagagtacaaactggtcgtggtgggggctgtgggtgtgggcaagtccgccctgactatccaactgatacagaaccatttcgtagatgaa

SEQ ID NO: 237 - RNA, 24 nt, synthetic construct
  source 1..24: mol_type = other RNA
gtcggcgcagtcggggtaggtaaa

SEQ ID NO: 238 - RNA, 93 nt, synthetic construct
  source 1..93: mol_type = other RNA
atgactgagtataaactcgtggttgtgggtgcagatggagtaggaaagagtgccctcacaatacaactgattcagaatcattttgtcgatgaa

SEQ ID NO: 239 - RNA, 24 nt, synthetic construct
  source 1..24: mol_type = other RNA
gtgggagctgatggtgttggcaag

SEQ ID NO: 240 - RNA, 93 nt, synthetic construct
  source 1..93: mol_type = other RNA
acctgcctgctggacatcctggacaccgcggggcacgaagagtatagcgctatgcgggaccagtacatgagaaccggtgagggctttctgtgt

SEQ ID NO: 241 - RNA, 24 nt, synthetic construct
  source 1..24: mol_type = other RNA
acagccggccacgaggagtattct

SEQ ID NO: 242 - RNA, 93 nt, synthetic construct
  source 1..93: mol_type = other RNA
actgagtacaagctggtggtggttggcgctggctgtgtggggaaatctgcattaacgattcaactgatccagaatcacttcgtcgatgagtac

SEQ ID NO: 243 - RNA, 24 nt, synthetic construct
  source 1..24: mol_type = other RNA
ggcgcaggctgcgtgggcaagtca

SEQ ID NO: 244 - RNA, 93 nt, synthetic construct
  source 1..93: mol_type = other RNA
acagagtacaagctggttgtcgttggggcaggggacgtcgggaagtccgccctgactatccagctgattcagaaccattttgtggacgaatat

SEQ ID NO: 245 - RNA, 24 nt, synthetic construct
  source 1..24: mol_type = other RNA
ggtgctggagacgtgggaaaatcc

SEQ ID NO: 246 - RNA, 93 nt, synthetic construct
  source 1..93: mol_type = other RNA
atgacagagtacaaacttgtggtggttggcgctgctggagtaggaaaatccgccctgaccatacaacttattcagaatcacttcgtggacgag

SEQ ID NO: 247 - RNA, 24 nt, synthetic construct
  source 1..24: mol_type = other RNA
gtcggggcggccggggtggggaag

SEQ ID NO: 248 - RNA, 93 nt, synthetic construct
  source 1..93: mol_type = other RNA
atgactgaatacaagttggtggtggtgggcgcgagcggggtgggtaagtctgccttgaccatccagctgatccagaaccatttcgttgatgaa

SEQ ID NO: 249 - RNA, 24 nt, synthetic construct
  source 1..24: mol_type = other RNA
gtcggcgcctcgggcgtggggaaa

SEQ ID NO: 250 - RNA, 93 nt, synthetic construct
  source 1..93: mol_type = other RNA
atgacagagtacaaactggtagtagtgggagcagatggggttggcaaatccgcgctcaccatccagctgattcaaaaccatttcgtcgatgag

SEQ ID NO: 251 - RNA, 24 nt, synthetic construct
  source 1..24: mol_type = other RNA
gtgggcgctgacggggtgggcaag

SEQ ID NO: 252 - RNA, 93 nt, synthetic construct
  source 1..93: mol_type = other RNA
atgaccgagtataaactcgtagtggtcggagctgtgggagtgggaaagtcagcgctcactatccaactaatacagaatcactttgtcgacgaa

SEQ ID NO: 253 - RNA, 24 nt, synthetic construct
  source 1..24: mol_type = other RNA
gtgggcgccgtgggtgtcggcaag

SEQ ID NO: 254 - RNA, 93 nt, synthetic construct
  source 1..93: mol_type = other RNA
atgacagaatacaagttggtcgttgttggtgcccgcggagtgggcaaatctgcactgaccatccaactgatccagaaccactttgtggatgag

SEQ ID NO: 255 - RNA, 24 nt, synthetic construct
  source 1..24: mol_type = other RNA
gtcggtgccaggggtgtgggaaag

SEQ ID NO: 256 - RNA, 93 nt, synthetic construct
  source 1..93: mol_type = other RNA
acatgtttgttagacattctcgacacggctgggcatgaggagtatagcgctatgcgggatcagtatatgagaaccggcgaaggctttctctgc

SEQ ID NO: 257 - RNA, 24 nt, synthetic construct
  source 1..24: mol_type = other RNA
acagccgggcacgaggaatattcc

SEQ ID NO: 258 - RNA, 93 nt, synthetic construct
  source 1..93: mol_type = other RNA
acttgcttgctggacatattagacacagcagggagggaagagtattccgcaatgcgagatcagtacatgcgtactggggaagggttcctgtgc

SEQ ID NO: 259 - RNA, 24 nt, synthetic construct
  source 1..24: mol_type = other RNA
accgccgggagggaggaatacagc

SEQ ID NO: 260 - RNA, 93 nt, synthetic construct
  source 1..93: mol_type = other RNA
actgagtacaagctggttgtggtgggagccggatgtgtcggtaaaagtgccctaaccatccagctcattcagaaccacttcgtcgatgagtat

SEQ ID NO: 261 - RNA, 93 nt, synthetic construct
  source 1..93: mol_type = other RNA
atgactgagtacaagctcgttgtcgtgggtgcatgcggagtagggaagtcagcgctgacaattcagttaatccagaatcacttcgtcgatgaa

SEQ ID NO: 262 - RNA, 24 nt, synthetic construct
  source 1..24: mol_type = other RNA
ggggccggctgtgttgggaaaagc

SEQ ID NO: 263 - RNA, 24 nt, synthetic construct
  source 1..24: mol_type = other RNA
gtcggcgcctgtggagtgggtaag

SEQ ID NO: 264 - RNA, 93 nt, synthetic construct
  source 1..93: mol_type = other RNA
acggagtacaagctggtcgtggttggcgccggcgacgtgggcaaaagcgctttgaccattcaactgatccagaatcattttgtggatgaatac

SEQ ID NO: 265 - RNA, 24 nt, synthetic construct
  source 1..24: mol_type = other RNA
ggggcaggggacgtggggaaatct

SEQ ID NO: 266 - RNA, 93 nt, synthetic construct
  source 1..93: mol_type = other RNA
atgactgaatataaattagttgtggtgggagccgatggagtggggaaatccgcgttgacaatccagctgatccagaaccattttgttgacgaa

SEQ ID NO: 267 - RNA, 24 nt, synthetic construct
  source 1..24: mol_type = other RNA
gttggagctgatggcgttggcaag

SEQ ID NO: 268 - RNA, 93 nt, synthetic construct
  source 1..93: mol_type = other RNA
atgacggaatacaagctggtcgtcgtgggcgcggtcggggtaggtaagtccgcgctgacaattcagctgattcagaatcacttcgtggatgag

SEQ ID NO: 269 - RNA, 24 nt, synthetic construct
  source 1..24: mol_type = other RNA
gtgggcgccgtgggagtcggtaag

SEQ ID NO: 270 - RNA, 93 nt, synthetic construct
  source 1..93: mol_type = other RNA
accgagtacaagctcgtggttgtcggtgctggtgacgtgggcaagtcggctctgacgatccaactgatccagaatcatttcgttgatgagtac

SEQ ID NO: 271 - RNA, 24 nt, synthetic construct
  source 1..24: mol_type = other RNA
ggggccggagatgtcggcaaatct

SEQ ID NO: 272 - RNA, 93 nt, synthetic construct
  source 1..93: mol_type = other RNA
aggtcatacgggatacctttcattgagacttccaccaaaactcgtcaacgcgtcgaggatgccttttataccctagtgagagagatccgacag

SEQ ID NO: 273 - RNA, 24 nt, synthetic construct
  source 1..24: mol_type = other RNA
gaaacaagcaccaagacccggcag

SEQ ID NO: 274 - RNA, 93 nt, synthetic construct
  source 1..93: mol_type = other RNA
atgacagaatacaagttggtagttgtcggcgcctgcggggtggggaaaagtgctctaaccattcaattaatccaaaatcactttgtcgacgag

SEQ ID NO: 275 - RNA, 24 nt, synthetic construct
  source 1..24: mol_type = other RNA
gtgggcgcctgcggggtaggcaaa

SEQ ID NO: 276 - RNA, 93 nt, synthetic construct
  source 1..93: mol_type = other RNA
atgaccgaatataaactggtggtggtgggagctgcaggagttggaaaaagcgctctgactatccaactgattcagaaccatttcgtggacgag

SEQ ID NO: 277 - RNA, 24 nt, synthetic construct
  source 1..24: mol_type = other RNA
gtcggggcagccggcgtgggaaaa

SEQ ID NO: 278 - RNA, 93 nt, synthetic construct
  source 1..93: mol_type = other RNA
atgaccgaatacaagctggtggtggttggcgcatccggtgtgggaaagtcagccctgacaatccagcttatacagaaccacttcgtcgacgaa

SEQ ID NO: 279 - RNA, 24 nt, synthetic construct
  source 1..24: mol_type = other RNA
gtgggcgcatctggagtcggaaag

SEQ ID NO: 280 - RNA, 93 nt, synthetic construct
  source 1..93: mol_type = other RNA
acagagtataaattggtggtggtaggtgctggatgtgtcggcaagtccgcacttactatacagctcattcagaaccactttgtagacgagtat

SEQ ID NO: 281 - RNA, 24 nt, synthetic construct
  source 1..24: mol_type = other RNA
ggggcagggtgcgtaggcaagtcc

SEQ ID NO: 282 - RNA, 93 nt, synthetic construct
  source 1..93: mol_type = other RNA
atgacggaatataagttggtcatggtgggtgcggatggtgtaggcaaatcagctctgactatccaactgatccagaatcactttgtggacgaa

SEQ ID NO: 283 - RNA, 24 nt, synthetic construct
  source 1..24: mol_type = other RNA
gtcggggctgacggtgtcggaaaa

SEQ ID NO: 284 - RNA, 93 nt, synthetic construct
  source 1..93: mol_type = other RNA
atgaccgaatataagctcgttgtggtgggggcttgtggagttggcaagtccgctctgactatccaactaattcagaatcatttcgtcgatgag

SEQ ID NO: 285 - RNA, 24 nt, synthetic construct
  source 1..24: mol_type = other RNA
gtcggcgcttgcggagtaggcaaa

SEQ ID NO: 286 - RNA, 93 nt, synthetic construct
  source 1..93: mol_type = other RNA
atgaccgaatacaagctcgtggtggtaggcgccgttggtgtagggaagagtgcgctaaccattcaacttatccagaaccattttgttgacgag

SEQ ID NO: 287 - RNA, 24 nt, synthetic construct
  source 1..24: mol_type = other RNA
gtaggcgcggtgggagtgggcaag

SEQ ID NO: 288 - RNA, 93 nt, synthetic construct
  source 1..93: mol_type = other RNA
atgaccgagtataaacttgtagtggtgggcgccaggggcgtggggaaaagcgccctgacaatccagctcatacagaatcacttcgtagacgag

SEQ ID NO: 289 - RNA, 24 nt, synthetic construct
  source 1..24: mol_type = other RNA
gtgggcgcccgcggcgttggtaag

SEQ ID NO: 290 - RNA, 93 nt, synthetic construct
  source 1..93: mol_type = other RNA
actgaatataaactcgtcgtcgtgggagcaggctgtgtggggaagagtgccttgaccattcagttgatccagaaccacttcgtcgacgagtat

SEQ ID NO: 291 - RNA, 24 nt, synthetic construct
  source 1..24: mol_type = other RNA
ggagcagggtgcgttggaaagagc

SEQ ID NO: 292 - RNA, 93 nt, synthetic construct
  source 1..93: mol_type = other RNA
acagaatacaaactggttgtcgtgggggccggcgacgtgggcaagagcgccttgactattcaactcatacagaaccactttgtggatgagtac

SEQ ID NO: 293 - RNA, 24 nt, synthetic construct
  source 1..24: mol_type = other RNA
ggcgccggggacgtggggaaaagc

SEQ ID NO: 294 - RNA, 93 nt, synthetic construct
  source 1..93: mol_type = other RNA
acgtgtcttctggatattttagacaccgcagggcatgaggagtactccgcaatgcgagatcagtacatgaggacaggtgagggtttcctgtgc

SEQ ID NO: 295 - RNA, 24 nt, synthetic construct
  source 1..24: mol_type = other RNA
acagccggccacgaggaatactct

SEQ ID NO: 296 - RNA, 797 nt, synthetic construct
  source 1..797: mol_type = other RNA
aagctttaatacgactcactataagtcctccccatcctctccctctgtccctctgtccctctgaccctgcactgtcccagcaccatggatatgagggtgcccgcccagctgctggggctgctgctgctgtggctgcggggcgcccggtgctacaagctggtcgtcgtgggggcctgcggcgtggggaagtccgctctgacctacaaactggtggtggtgggggccgatggggtgggcaagtccgccctgacctacaagctggtggtggtcggggccgtcggcgtgggcaaaagcgccctgacatacaagctcgtggtggtgggcgccaggggggtgggcaagtccgccctgacaaagctggtcgtggtgggcgccgggtgcgtgggcaagagcgccctgacaatcaagctggtggtggtgggggccggggatgtgggcaagagcgccctgaccatcctggacatcctggacacagccgggcacgaggagtacagcgccatgagggattgatgactcgaggtgtgtggaggacaccctgaaccccccgctttcaaacaagttttcaaattgtttgaggtcaggatttctcaaactgattcctttctttgcatatgagtatttgaaaataaatattttcccagaatataaataaatcatcacatgattattttaactatgctagcaaaaaaaaaaaaaaaaaaaaaaaaaaaaaaaaaaaaaaaaaaaaaaaaaaaaaaaaaaaaaaaaaaaaaaaaaaaaaaaaaaaaaaaaaaaaaaaaaaaaagaagagcgaattc

SEQ ID NO: 297 - RNA, 881 nt, synthetic construct
  source 1..881: mol_type = other RNA
aagctttaatacgactcactataagtcctccccatcctctccctctgtccctctgtccctctgaccctgcactgtcccagcaccatggatatgagagtgcccgcccaactgctggggctgctgctgctgtggctgagaggcgcgagatgcatgacagaatacaaacttgtggtagttggagcatgcggtgtgggtaagagtgccctcaccatccaactaattcagaaccacttcgttgacgaactcctctcagtggggggggttggagcatgtggtgtagggaagctgttgagcgtcggcgggatgactgaatacaaacttgtggttgttggagcagatggggtcggaaaatccgccttgacaatacagcttattcagaatcactttgtggatgagctgttaagcgttggcggcgtcggagctgatggcgtcggaaagctcttgtctgtgggcggcactgagtataaattagtggtagtcggggctggagacgtgggcaagagtgcccttaccatccagctcatccagaatcattttgtggacgagtatctattgtccgtgggaggtggagctggtgacgtcggaaagtcttaatgactcgaggtgtgtggaggacaccctgaaccccccgctttcaaacaagttttcaaattgtttgaggtcaggatttctcaaactgattcctttctttgcatatgagtatttgaaaataaatattttcccagaatataaataaatcatcacatgattattttaactatgctagcaaaaaaaaaaaaaaaaaaaaaaaaaaaaaaaaaaaaaaaaaaaaaaaaaaaaaaaaaaaaaaaaaaaaaaaaaaaaaaaaaaaaaaaaaaaaaaaaaaaaagaagagcgaattc

SEQ ID NO: 298 - RNA, 1365 nt, synthetic construct
  source 1..1365: mol_type = other RNA
aagctttaatacgactcactataagaatccagtcaacgcatatccacgtatacccgaacacatcacagccaccatggatatgcgagtgcccgctcagcttctggggttgcttctgttatggctgaggggggcccggtgtatgacagaatacaagttagtggtggtaggagcgtgtggagtggggaaaagcgccctaactattcagttgatacaaaaccatttcgtggacgaagtgggcgcatgtggagtcggcaagatgaccgagtataagctcgtagtcgtgggggccgacggcgtggggaaatcagcccttactatccagcttatacaaaaccattttgttgacgaagtaggcgccgacggggtcggaaagatgaccgagtacaagctggttgtcgtcggggccgtaggggttggcaaaagcgccctgactatccagctcatccaaaatcatttcgtcgacgaggtgggcgccgttggagtcggtaaaatgacggaatacaagttggtggtagtgggggctcggggggtgggcaagagtgctttgaccatacagttaattcagaaccactttgtggatgaggtcggcgctcgcggagtcggcaaaaccgagtataaattggttgttgtcggcgcaggctgtgtgggcaagtctgctctcaccattcaactaatccagaaccactttgttgatgagtacggagcaggctgcgtgggaaaaagcacggagtacaagctggttgtcgtaggagcaggagacgtgggcaaatccgctctgacaattcagcttatccagaatcactttgtggatgaatatggtgccggggatgtcggtaaaagtacctgcttactggacatcctggacactgctggtcacgaggaatactccgcgatgcgagatcagtatatgcggacaggagagggtttcctgtgcacagcaggccatgaggaatattctactgaatataagctggtggtggtgggggctggtagagtggggaagtcagcactgacaatccagctcattcagaatcacttcgttgatgagtacggtgcgggtagagtgggcaagtcctaatgactcgaggtgtgtggaggacaccctgaaccccccgctttcaaacaagttttcaaattgtttgaggtcaggatttctcaaactgattcctttctttgcatatgagtatttgaaaataaatattttcccagaatataaataaatcatcacatgattattttaactatgctagcaaaaaaaaaaaaaaaaaaaaaaaaaaaaaaaaaaaaaaaaaaaaaaaaaaaaaaaaaaaaaaaaaaaaaaaaaaaaaaaaaaaaaaaaaaaaaaaaaaaaagaagagcgaattc

SEQ ID NO: 299 - RNA, 1635 nt, synthetic construct
  source 1..1635: mol_type = other RNA
aagctttaatacgactcactataagaatccagtcaacgcatatccacgtatacccgaacacatcacagccaccatggatatgcgagtgcccgctcagcttctggggttgcttctgttatggctgaggggggcccggtgtatgacggaatacaagctcgtcgtggtgggcgccgatggcgtcggcaagtcggcactgactatccagctcatacaaaatcattttgttgatgaacttttatccgtcggtggagtgggggcggacggagtggggaagctgctgagcgttggtgggatgaccgaatacaaactggtggtggtcggggcgtgtggggtgggcaaatcagccctcacaatacagctgattcagaaccactttgttgacgagcttctgtccgtgggcggggtgggggcatgtggagtggggaagctcctgtccgtagggggcatgactgagtacaagctggttgttgtaggtgctgttggagtgggaaagagcgccctcacaatccaattgatccagaatcacttcgtcgacgagctcttgagcgttggaggtgtgggggccgtaggcgtgggcaagctgctatctgtgggtggaatgaccgaatataagttggtagtggtgggggctcgcggagtcgggaagagtgctcttactattcagctgattcagaaccatttcgtagatgaactcctatcagtcggtggcgtgggcgccagaggcgtgggcaaactgttatcagtgggcggtactgagtacaaactagtagtcgtaggagctgggtgtgtgggcaaaagtgcactcaccatccagctgatccagaaccatttcgtggatgagtatttgttgagtgtcggaggtggagctggctgcgtgggcaaaagcctgctgtccgttggggggacggaatacaaactagttgttgtgggggctggtgatgtcggaaagtccgccttgactattcagcttattcaaaatcactttgtcgacgagtatcttctgagcgtcggcggcggcgcaggtgacgtaggaaagtctttactgtcagttgggggaacctgccttctggacatcctggacacagccggccacgaggaatacagcgccatgcgggatcagtatatgaggacaggagaaggcttcctctgcctcttaagtgtcggcggtacagctggccacgaggagtattctctgctgtctgtcggaggcaccgagtacaaacttgtggtggttggagcagggcgtgtcggcaaatctgccctgaccatccagctgatacaaaaccattttgtggatgagtatttactttccgtgggaggcggtgcgggacgagtgggcaagagctaatgactcgaggtgtgtggaggacaccctgaaccccccgctttcaaacaagttttcaaattgtttgaggtcaggatttctcaaactgattcctttctttgcatatgagtatttgaaaataaatattttcccagaatataaataaatcatcacatgattattttaactatgctagcaaaaaaaaaaaaaaaaaaaaaaaaaaaaaaaaaaaaaaaaaaaaaaaaaaaaaaaaaaaaaaaaaaaaaaaaaaaaaaaaaaaaaaaaaaaaaaaaaaaaagaagagcgaattc

SEQ ID NO: 300 - RNA, 1482 nt, synthetic construct
  source 1..1482: mol_type = other RNA
aagctttaatacgactcactataagaatccagtcaacgcatatccacgtatacccgaacacatcacagccaccatggacatgagggtgcccgcccagttgctggggctgctgctcttgtggctcagaggggcacggtgcatgacggaatacaagctcgtcgtggtgggcgccgatggcgtcggcaagtcggcactgactatccagctcatacaaaatcattttgttgatgaacttttatccgtcggtggagtgggggcggacggagtggggaagctgctgagcgttggtgggatgaccgaatacaaactggtggtggtcggggcgtgtggggtgggcaaatcagccctcacaatacagctgattcagaaccactttgttgacgagcttctgtccgtgggcggggtgggggcatgtggagtggggaagctcctgtccgtagggggcatgactgagtacaagctggttgttgtaggtgctgttggagtgggaaagagcgccctcacaatccaattgatccagaatcacttcgtcgacgagctcttgagcgttggaggtgtgggggccgtaggcgtgggcaagctgctatctgtgggtggaatgaccgaatataagttggtagtggtgggggctcgcggagtcgggaagagtgctcttactattcagctgattcagaaccatttcgtagatgaactcctatcagtcggtggcgtgggcgccagaggcgtgggcaaactgttatcagtgggcggtactgagtacaaactagtagtcgtaggagctgggtgtgtgggcaaaagtgcactcaccatccagctgatccagaaccatttcgtggatgagtatttgttgagtgtcggaggtggagctggctgcgtgggcaaaagcctgctgtccgttggggggacggaatacaaactagttgttgtgggggctggtgatgtcggaaagtccgccttgactattcagcttattcaaaatcactttgtcgacgagtatcttctgagcgtcggcggcggcgcaggtgacgtaggaaagtctttactgtcagttgggggaacctgccttctggacatcctggacacagccggccacgaggaatacagcgccatgcgggatcagtatatgaggacaggagaaggcttcctctgcctcttaagtgtcggcggtacagctggccacgaggagtattcttaatgactcgaggtgtgtggaggacaccctgaaccccccgctttcaaacaagttttcaaattgtttgaggtcaggatttctcaaactgattcctttctttgcatatgagtatttgaaaataaatattttcccagaatataaataaatcatcacatgattattttaactatgctagcaaaaaaaaaaaaaaaaaaaaaaaaaaaaaaaaaaaaaaaaaaaaaaaaaaaaaaaaaaaaaaaaaaaaaaaaaaaaaaaaaaaaaaaaaaaaaaaaaaaaagaagagcgaattc

SEQ ID NO: 301 - protein, 23 aa, synthetic construct
MTEYKLVVVGARGVGKSALTIQL

SEQ ID NO: 302 - protein, 19 aa, synthetic construct
EYKLVVVGADGVGKSALTI

SEQ ID NO: 303 - protein, 19 aa, synthetic construct
EYKLVVVGAVGVGKSALTI

SEQ ID NO: 304 - protein, 19 aa, synthetic construct
EYKLVVVGACGVGKSALTI

SEQ ID NO: 305 - protein, 19 aa, synthetic construct
YKLVVVGAGDVGKSALTIQ

SEQ ID NO: 306 - protein, 19 aa, synthetic construct
YKLVVVGAGCVGKSALTIQ

SEQ ID NO: 307 - protein, 19 aa, synthetic construct
LLDILDTAGHEEYSAMRDQ

SEQ ID NO: 308 - protein, 17 aa, synthetic construct
YKLVVVGACGVGKSALT

SEQ ID NO: 309 - protein, 17 aa, synthetic construct
YKLVVVGADGVGKSALT

SEQ ID NO: 310 - protein, 17 aa, synthetic construct
YKLVVVGAVGVGKSALT

SEQ ID NO: 311 - protein, 17 aa, synthetic construct
YKLVVVGARGVGKSALT

SEQ ID NO: 312 - protein, 17 aa, synthetic construct
KLVVVGAGCVGKSALTI

SEQ ID NO: 313 - protein, 17 aa, synthetic construct
KLVVVGAGDVGKSALTI

SEQ ID NO: 314 - protein, 17 aa, synthetic construct
LDILDTAGHEEYSAMRD

SEQ ID NO: 315 - protein, 17 aa, synthetic construct
YKLVVVGACGVGKSALT

SEQ ID NO: 316 - protein, 17 aa, synthetic construct
YKLVVVGADGVGKSALT

SEQ ID NO: 317 - protein, 17 aa, synthetic construct
YKLVVVGAVGVGKSALT

SEQ ID NO: 318 - protein, 17 aa, synthetic construct
YKLVVVGARGVGKSALT

SEQ ID NO: 319 - protein, 17 aa, synthetic construct
KLVVVGAGCVGKSALTI

SEQ ID NO: 320 - protein, 17 aa, synthetic construct
KLVVVGAGDVGKSALTI

SEQ ID NO: 321 - protein, 17 aa, synthetic construct
LDILDTAGHEEYSAMRD

SEQ ID NO: 322 - protein, 9 aa, synthetic construct
VGACGVGKS

SEQ ID NO: 323 - protein, 9 aa, synthetic construct
VVVGACGVG

SEQ ID NO: 324 - protein, 9 aa, synthetic construct
VGACGVGKS

SEQ ID NO: 325 - protein, 9 aa, synthetic construct
VVVGACGVG

SEQ ID NO: 326 - protein, 9 aa, synthetic construct
VGACGVGKS

SEQ ID NO: 327 - protein, 9 aa, synthetic construct
VVVGACGVG

SEQ ID NO: 328 - protein, 9 aa, synthetic construct
VGACGVGKS

SEQ ID NO: 329 - protein, 9 aa, synthetic construct
VVVGACGVG

SEQ ID NO: 330 - protein, 9 aa, synthetic construct
VGADGVGKS

SEQ ID NO: 331 - protein, 9 aa, synthetic construct
VVVGADGVG

SEQ ID NO: 332 - protein, 9 aa, synthetic construct
GAGDVGKSA

SEQ ID NO: 333 - protein, 9 aa, synthetic construct
VVGAGDVGK

SEQ ID NO: 334 - protein, 31 aa, synthetic construct
MTEYKLVVVGACGVGKSALTIQLIQNHFVDE

SEQ ID NO: 335 - protein, 8 aa, synthetic construct
VGACGVGK

SEQ ID NO: 336 - protein, 31 aa, synthetic construct
MTEYKLVVVGADGVGKSALTIQLIQNHFVDE

SEQ ID NO: 337 - protein, 8 aa, synthetic construct
VGADGVGK

SEQ ID NO: 338 - protein, 31 aa, synthetic construct
TEYKLVVVGAGDVGKSALTIQLIQNHFVDEY

SEQ ID NO: 339 - protein, 8 aa, synthetic construct
GAGDVGKS

SEQ ID NO: 340 - protein, 31 aa, synthetic construct
MTEYKLVVVGAGCVGKSALTIQLIQNHFVDE

SEQ ID NO: 341 - protein, 31 aa, synthetic construct; identical to SEQ ID NO: 334

SEQ ID NO: 342 - protein, 31 aa, synthetic construct; identical to SEQ ID NO: 336

SEQ ID NO: 343 - protein, 31 aa, synthetic construct
MTEYKLVVVGAGDVGKSALTIQLIQNHFVDE

SEQ ID NO: 344 - protein, 31 aa, synthetic construct
MTEYKLVVVGAVGVGKSALTIQLIQNHFVDE

SEQ ID NO: 345 - protein, 31 aa, synthetic construct
TCLLDILDTAGHEEYSAMRDQYMRTGEGFLC

SEQ ID NO: 346 - protein, 31 aa, synthetic construct; identical to SEQ ID NO: 334

SEQ ID NO: 347 - protein, 8 aa, synthetic construct
VGACGVGK

SEQ ID NO: 348 - protein, 31 aa, synthetic construct; identical to SEQ ID NO: 336

SEQ ID NO: 349 - protein, 8 aa, synthetic construct
VGADGVGK

SEQ ID NO: 350 - protein, 31 aa, synthetic construct; identical to SEQ ID NO: 338

SEQ ID NO: 351 - protein, 8 aa, synthetic construct
GAGDVGKS

SEQ ID NO: 352 - protein, 177 aa, synthetic construct
CINLDWDVIRDKTKTKIESLKEHGPIKNKMSESPNKTVSEEKAKQYLEEFHQTALEHPELSELKTVTGTNPVFAGANYAAWAVNVAQVIDSETADNLEKTTAALSILPGIGSVMGIADGAVHHNTEEIVAQSIALSSLMVAQAIPLVGELVDIGFAAYNFVESIINLFQVVHNSYNR

SEQ ID NO: 353 - protein, 31 aa, synthetic construct; identical to SEQ ID NO: 340

SEQ ID NO: 354 - protein, 31 aa, synthetic construct; identical to SEQ ID NO: 334

SEQ ID NO: 355 - protein, 31 aa, synthetic construct; identical to SEQ ID NO: 336

SEQ ID NO: 356 - protein, 31 aa, synthetic construct; identical to SEQ ID NO: 343

SEQ ID NO: 357 - protein, 31 aa, synthetic construct; identical to SEQ ID NO: 344

SEQ ID NO: 358 - protein, 31 aa, synthetic construct; identical to SEQ ID NO: 345

SEQ ID NO: 359 - protein, 31 aa, synthetic construct; identical to SEQ ID NO: 340

SEQ ID NO: 360 - protein, 31 aa, synthetic construct; identical to SEQ ID NO: 334

SEQ ID NO: 361 - protein, 31 aa, synthetic construct; identical to SEQ ID NO: 336

SEQ ID NO: 362 - protein, 31 aa, synthetic construct; identical to SEQ ID NO: 343

SEQ ID NO: 363 - protein, 31 aa, synthetic construct; identical to SEQ ID NO: 344

SEQ ID NO: 364 - protein, 31 aa, synthetic construct; identical to SEQ ID NO: 345

SEQ ID NO: 365 - protein, 177 aa, synthetic construct; identical to SEQ ID NO: 352

SEQ ID NO: 366 - protein, 87 aa, synthetic construct
CINLDWDVIRDKTKTKIESLKEHGPIKNKMSESPNKTVSEEKAKQYLEEFHQTALEHPELSELKTVTGTNPVFAGANYAAWAVNVAQ

SEQ ID NO: 367 - protein, 31 aa, synthetic construct; identical to SEQ ID NO: 340

SEQ ID NO: 368 - protein, 31 aa, synthetic construct; identical to SEQ ID NO: 334

SEQ ID NO: 369 - protein, 31 aa, synthetic construct; identical to SEQ ID NO: 336

SEQ ID NO: 370 - protein, 31 aa, synthetic construct; identical to SEQ ID NO: 343

SEQ ID NO: 371 - protein, 31 aa, synthetic construct; identical to SEQ ID NO: 344

SEQ ID NO: 372 - protein, 31 aa, synthetic construct; identical to SEQ ID NO: 345

SEQ ID NO: 373 - protein, 82 aa, synthetic construct
NLEKTTAALSILPGIGSVMGIADGAVHHNTEEIVAQSIALSSLMVAQAIPLVGELVDIGFAAYNFVESIINLFQVVHNSYNR

SEQ ID NO: 374 - protein, 31 aa, synthetic construct; identical to SEQ ID NO: 345

SEQ ID NO: 375 - protein, 17 aa, synthetic construct
YKLVVVGACGVGKSALT

SEQ ID NO: 376 - protein, 17 aa, synthetic construct
YKLVVVGADGVGKSALT

SEQ ID NO: 377 - protein, 17 aa, synthetic construct
YKLVVVGARGVGKSALT

SEQ ID NO: 378 - protein, 17 aa, synthetic construct
YKLVVVGAVGVGKSALT

SEQ ID NO: 379 - protein, 17 aa, synthetic construct
KLVVVGAGCVGKSALTI

SEQ ID NO: 380 - protein, 17 aa, synthetic construct
LDILDTAGHEEYSAMRD

SEQ ID NO: 381 - protein, 17 aa, synthetic construct
KLVVVGAGDVGKSALTI

SEQ ID NO: 382 - protein, 17 aa, synthetic construct
KLVVVGAGRVGKSALTI

SEQ ID NO: 383 - protein, 31 aa, synthetic construct; identical to SEQ ID NO: 334

SEQ ID NO: 384 - protein, 8 aa, synthetic construct
VGACGVGK

SEQ ID NO: 385 - protein, 31 aa, synthetic construct; identical to SEQ ID NO: 336

SEQ ID NO: 386 - protein, 8 aa, synthetic construct
VGADGVGK

SEQ ID NO: 387 - protein, 31 aa, synthetic construct; identical to SEQ ID NO: 344

SEQ ID NO: 388 - protein, 8 aa, synthetic construct
VGAVGVGK

SEQ ID NO: 389 - protein, 31 aa, synthetic construct
MTEYKLVVVGARGVGKSALTIQLIQNHFVDE

SEQ ID NO: 390 - protein, 8 aa, synthetic construct
VGARGVGK

SEQ ID NO: 391 - protein, 31 aa, synthetic construct
TEYKLVVVGAGCVGKSALTIQLIQNHFVDEY

SEQ ID NO: 392 - protein, 8 aa, synthetic construct
GAGCVGKS

SEQ ID NO: 393 - protein, 31 aa, synthetic construct; identical to SEQ ID NO: 338

SEQ ID NO: 394 - protein, 8 aa, synthetic construct
GAGDVGKS

SEQ ID NO: 395 - protein, 8 aa, synthetic construct
TAGHEEYS

SEQ ID NO: 396 - protein, 31 aa, synthetic construct
TEYKLVVVGAGRVGKSALTIQLIQNHFVDEY

SEQ ID NO: 397 - protein, 8 aa, synthetic construct
GAGRVGKS

SEQ ID NO: 398 - protein, 31 aa, synthetic construct; identical to SEQ ID NO: 334

SEQ ID NO: 399 - protein, 8 aa, synthetic construct
VGACGVGK

SEQ ID NO: 400 - protein, 31 aa, synthetic construct; identical to SEQ ID NO: 336

SEQ ID NO: 401 - protein, 8 aa, synthetic construct
VGADGVGK

SEQ ID NO: 402 - protein, 31 aa, synthetic construct; identical to SEQ ID NO: 344

SEQ ID NO: 403 - protein, 8 aa, synthetic construct
VGAVGVGK

SEQ ID NO: 404 - protein, 31 aa, synthetic construct; identical to SEQ ID NO: 389

SEQ ID NO: 405 - protein, 8 aa, synthetic construct
VGARGVGK

SEQ ID NO: 406 - protein, 31 aa, synthetic construct; identical to SEQ ID NO: 391

SEQ ID NO: 407 - protein, 8 aa, synthetic construct
GAGCVGKS

SEQ ID NO: 408 - protein, 31 aa, synthetic construct; identical to SEQ ID NO: 338

SEQ ID NO: 409 - protein, 8 aa, synthetic construct
GAGDVGKS

SEQ ID NO: 410 - protein, 31 aa, synthetic construct; identical to SEQ ID NO: 345

SEQ ID NO: 411 - protein, 8 aa, synthetic construct
TAGHEEYS

SEQ ID NO: 412 - protein, 31 aa, synthetic construct; identical to SEQ ID NO: 396

SEQ ID NO: 413 - protein, 8 aa, synthetic construct
GAGRVGKS

SEQ ID NO: 414 - protein, 31 aa, synthetic construct; identical to SEQ ID NO: 336

SEQ ID NO: 415 - protein, 8 aa, synthetic construct
VGADGVGK

SEQ ID NO: 416 - protein, 31 aa, synthetic construct; identical to SEQ ID NO: 334

SEQ ID NO: 417 - protein, 8 aa, synthetic construct
VGACGVGK

SEQ ID NO: 418 - protein, 31 aa, synthetic construct; identical to SEQ ID NO: 344

SEQ ID NO: 419 - protein, 8 aa, synthetic construct
VGAVGVGK

SEQ ID NO: 420 - protein, 31 aa, synthetic construct; identical to SEQ ID NO: 389

SEQ ID NO: 421 - protein, 8 aa, synthetic construct
VGARGVGK

SEQ ID NO: 422 - protein, 31 aa, synthetic construct; identical to SEQ ID NO: 391

SEQ ID NO: 423 - protein, 8 aa, synthetic construct
GAGCVGKS

SEQ ID NO: 424 - protein, 31 aa, synthetic construct; identical to SEQ ID NO: 344

SEQ ID NO: 425 - protein, 31 aa, synthetic construct; identical to SEQ ID NO: 338

SEQ ID NO: 426 - protein, 8 aa, synthetic construct
GAGDVGKS

SEQ ID NO: 427 - protein, 31 aa, synthetic construct; identical to SEQ ID NO: 345

SEQ ID NO: 428 - protein, 31 aa, synthetic construct; identical to SEQ ID NO: 344

SEQ ID NO: 429 - protein, 8 aa, synthetic construct
TAGHEEYS

SEQ ID NO: 430 - protein, 31 aa, synthetic construct; identical to SEQ ID NO: 396

SEQ ID NO: 431 - protein, 8 aa, synthetic construct
GAGRVGKS

SEQ ID NO: 432 - protein, 17 aa, synthetic construct
YKLVVVGACGVGKSALT

SEQ ID NO: 433 - protein, 17 aa, synthetic construct
YKLVVVGADGVGKSALT

SEQ ID NO: 434 - protein, 17 aa, synthetic construct
YKLVVVGAVGVGKSALT

SEQ ID NO: 435 - protein, 17 aa, synthetic construct
YKLVVVGARGVGKSALT

SEQ ID NO: 436 - protein, 17 aa, synthetic construct
KLVVVGAGCVGKSALTI

SEQ ID NO: 437 - protein, 17 aa, synthetic construct
KLVVVGAGDVGKSALTI

SEQ ID NO: 438 - protein, 17 aa, synthetic construct
LDILDTAGHEEYSAMRD

SEQ ID NO: 439 - protein, 17 aa, synthetic construct
KLVVVGAGRVGKSALTI

SEQ ID NO: 440 - protein, 17 aa, synthetic construct
YKLVVVGACGVGKSALT

SEQ ID NO: 441 - protein, 17 aa, synthetic construct
YKLVVVGADGVGKSALT

SEQ ID NO: 442 - protein, 17 aa, synthetic construct
YKLVVVGAVGVGKSALT

SEQ ID NO: 443 - protein, 17 aa, synthetic construct
YKLVVVGARGVGKSALT

SEQ ID NO: 444 - protein, 17 aa, synthetic construct
KLVVVGAGCVGKSALTI

SEQ ID NO: 445 - protein, 17 aa, synthetic construct
LDILDTAGHEEYSAMRD

SEQ ID NO: 446 - protein, 17 aa, synthetic construct
KLVVVGAGDVGKSALTI

SEQ ID NO: 447 - protein, 17 aa, synthetic construct
KLVVVGAGRVGKSALTI

SEQ ID NO: 448 - protein, 17 aa, synthetic construct
YKLVVVGAVGVGKSALT

SEQ ID NO: 449 - protein, 17 aa, synthetic construct
YKLVVVGARGVGKSALT

SEQ ID NO: 450 - protein, 17 aa, synthetic construct
KLVVVGAGCVGKSALTI

SEQ ID NO: 451 - protein, 17 aa, synthetic construct
LDILDTAGHEEYSAMRD

SEQ ID NO: 452 - protein, 17 aa, synthetic construct
YKLVVVGACGVGKSALT

SEQ ID NO: 453 - protein, 17 aa, synthetic construct
YKLVVVGADGVGKSALT

SEQ ID NO: 454 - protein, 17 aa, synthetic construct
KLVVVGAGDVGKSALTI

SEQ ID NO: 455 - protein, 17 aa, synthetic construct
KLVVVGAGRVGKSALTI

SEQ ID NO: 456 - protein, 31 aa, synthetic construct; identical to SEQ ID NO: 336

SEQ ID NO: 457 - protein, 8 aa, synthetic construct
VGADGVGK

SEQ ID NO: 458 - protein, 31 aa, synthetic construct; identical to SEQ ID NO: 334

SEQ ID NO: 459 - protein, 8 aa, synthetic construct
VGACGVGK

SEQ ID NO: 460 - protein, 31 aa, synthetic construct; identical to SEQ ID NO: 344

SEQ ID NO: 461 - protein, 8 aa, synthetic construct
VGAVGVGK

SEQ ID NO: 462 - protein, 31 aa, synthetic construct; identical to SEQ ID NO: 389

SEQ ID NO: 463 - protein, 8 aa, synthetic construct
VGARGVGK

SEQ ID NO: 464 - protein, 31 aa, synthetic construct; identical to SEQ ID NO: 391

SEQ ID NO: 465 - protein, 8 aa, synthetic construct
GAGCVGKS

SEQ ID NO: 466 - protein, 31 aa, synthetic construct; identical to SEQ ID NO: 338

SEQ ID NO: 467 - protein, 8 aa, synthetic construct
GAGDVGKS

SEQ ID NO: 468 - protein, 31 aa, synthetic construct; identical to SEQ ID NO: 345

SEQ ID NO: 469 - protein, 8 aa, synthetic construct
TAGHEEYS

SEQ ID NO: 470 - protein, 31 aa, synthetic construct; identical to SEQ ID NO: 336

SEQ ID NO: 471 - protein, 8 aa, synthetic construct
VGADGVGK

SEQ ID NO: 472 - protein, 31 aa, synthetic construct; identical to SEQ ID NO: 334

SEQ ID NO: 473 - protein, 8 aa, synthetic construct
VGACGVGK

SEQ ID NO: 474 - protein, 8 aa, synthetic construct
VGAVGVGK

SEQ ID NO: 475 - protein, 31 aa, synthetic construct; identical to SEQ ID NO: 389

SEQ ID NO: 476 - protein, 8 aa, synthetic construct
VGARGVGK

SEQ ID NO: 477 - protein, 31 aa, synthetic construct; identical to SEQ ID NO: 345

SEQ ID NO: 478 - protein, 8 aa, synthetic construct
TAGHEEYS

SEQ ID NO: 479 - protein, 31 aa, synthetic construct; identical to SEQ ID NO: 338

SEQ ID NO: 480 - protein, 8 aa, synthetic construct
GAGDVGKS

SEQ ID NO: 481 - protein, 31 aa, synthetic construct
MTEYKLVVVGAAGVGKSALTIQLIQNHFVDE

SEQ ID NO: 482 - protein, 8 aa, synthetic construct
VGAAGVGK

SEQ ID NO: 483 - protein, 31 aa, synthetic construct
RSYGIPFIETSTKTRQRVEDAFYTLVREIRQ

SEQ ID NO: 484 - protein, 8 aa, synthetic construct
ETSTKTRQ

SEQ ID NO: 485 - protein, 31 aa, synthetic construct; identical to SEQ ID NO: 391

SEQ ID NO: 486 - protein, 8 aa, synthetic construct
GAGCVGKS

SEQ ID NO: 487 - protein, 31 aa, synthetic construct
MTEYKLVVVGASGVGKSALTIQLIQNHFVDE

SEQ ID NO: 488 - protein, 8 aa, synthetic construct
VGASGVGK

SEQ ID NO: 489 - protein, 31 aa, synthetic construct
TCLLDILDTAGREEYSAMRDQYMRTGEGFLC

SEQ ID NO: 490 - protein, 8 aa, synthetic construct
TAGREEYS

SEQ ID NO: 491 - protein, 31 aa, synthetic construct; identical to SEQ ID NO: 334

SEQ ID NO: 492 - protein, 8 aa, synthetic construct
VGACGVGK

SEQ ID NO: 493 - protein, 31 aa, synthetic construct; identical to SEQ ID NO: 344

SEQ ID NO: 494 - protein, 8 aa, synthetic construct
VGAVGVGK

SEQ ID NO: 495 - protein, 31 aa, synthetic construct; identical to SEQ ID NO: 336

SEQ ID NO: 496 - protein, 8 aa, synthetic construct
VGADGVGK

SEQ ID NO: 497 - protein, 31 aa, synthetic construct; identical to SEQ ID NO: 345

SEQ ID NO: 498 - protein, 8 aa, synthetic construct
TAGHEEYS

SEQ ID NO: 499 - protein, 31 aa, synthetic construct; identical to SEQ ID NO: 391

SEQ ID NO: 500 - protein, 8 aa, synthetic construct
GAGCVGKS

SEQ ID NO: 501 - protein, 31 aa, synthetic construct; identical to SEQ ID NO: 338

SEQ ID NO: 502 - protein, 8 aa, synthetic construct
GAGDVGKS

SEQ ID NO: 503 - protein, 31 aa, synthetic construct; identical to SEQ ID NO: 481

SEQ ID NO: 504 - protein, 8 aa, synthetic construct
VGAAGVGK

SEQ ID NO: 505 - protein, 31 aa, synthetic construct; identical to SEQ ID NO: 487

SEQ ID NO: 506 - protein, 8 aa, synthetic construct
VGASGVGK

SEQ ID NO: 507 - protein, 31 aa, synthetic construct; identical to SEQ ID NO: 336

SEQ ID NO: 508 - protein, 8 aa, synthetic construct
VGADGVGK

SEQ ID NO: 509 - protein, 31 aa, synthetic construct; identical to SEQ ID NO: 344

SEQ ID NO: 510 - protein, 8 aa, synthetic construct
VGAVGVGK

SEQ ID NO: 511 - protein, 31 aa, synthetic construct; identical to SEQ ID NO: 389

SEQ ID NO: 512 - protein, 8 aa, synthetic construct
VGARGVGK

SEQ ID NO: 513 - protein, 31 aa, synthetic construct; identical to SEQ ID NO: 345

SEQ ID NO: 514 - protein, 8 aa, synthetic construct
TAGHEEYS

SEQ ID NO: 515 - protein, 31 aa, synthetic construct; identical to SEQ ID NO: 489

SEQ ID NO: 516 - protein, 8 aa, synthetic construct
TAGREEYS

SEQ ID NO: 517 - protein, 31 aa, synthetic construct; identical to SEQ ID NO: 391

SEQ ID NO: 518 - protein, 8 aa, synthetic construct
GAGCVGKS

SEQ ID NO: 519 - protein, 31 aa, synthetic construct; identical to SEQ ID NO: 334

SEQ ID NO: 520 - protein, 8 aa, synthetic construct
VGACGVGK

SEQ ID NO: 521 - protein, 31 aa, synthetic construct; identical to SEQ ID NO: 338

SEQ ID NO: 522 - protein, 8 aa, synthetic construct
GAGDVGKS

SEQ ID NO: 523 - protein, 31 aa, synthetic construct; identical to SEQ ID NO: 336

SEQ ID NO: 524 - protein, 8 aa, synthetic construct
VGADGVGK

SEQ ID NO: 525 - protein, 8 aa, synthetic construct
VGAVGVGK

SEQ ID NO: 526 - protein, 31 aa, synthetic construct; identical to SEQ ID NO: 338

SEQ ID NO: 527 - protein, 8 aa, synthetic construct
GAGDVGKS

SEQ ID NO: 528 - protein, 31 aa, synthetic construct; identical to SEQ ID NO: 483

SEQ ID NO: 529 - protein, 8 aa, synthetic construct
ETSTKTRQ

SEQ ID NO: 530 - protein, 31 aa, synthetic construct; identical to SEQ ID NO: 334

SEQ ID NO: 531 - protein, 8 aa, synthetic construct
VGACGVGK

SEQ ID NO: 532 - protein, 31 aa, synthetic construct; identical to SEQ ID NO: 481

SEQ ID NO: 533 - protein, 8 aa, synthetic construct
VGAAGVGK

SEQ ID NO: 534 - protein, 31 aa, synthetic construct; identical to SEQ ID NO: 487

SEQ ID NO: 535 - protein, 8 aa, synthetic construct
VGASGVGK

SEQ ID NO: 536 - protein, 31 aa, synthetic construct; identical to SEQ ID NO: 391

SEQ ID NO: 537 - protein, 8 aa, synthetic construct
GAGCVGKS

SEQ ID NO: 538 - protein, 31 aa, synthetic construct
MTEYKLVMVGADGVGKSALTIQLIQNHFVDE

SEQ ID NO: 539 - protein, 8 aa, synthetic construct
VGADGVGK

SEQ ID NO: 540 - protein, 31 aa, synthetic construct; identical to SEQ ID NO: 334

SEQ ID NO: 541 - protein, 8 aa, synthetic construct
VGACGVGK

SEQ ID NO: 542 - protein, 31 aa, synthetic construct; identical to SEQ ID NO: 344

SEQ ID NO: 543 - protein, 8 aa, synthetic construct
VGAVGVGK

SEQ ID NO: 544 - protein, 31 aa, synthetic construct; identical to SEQ ID NO: 389

SEQ ID NO: 545 - protein, 8 aa, synthetic construct
VGARGVGK

SEQ ID NO: 546 - protein, 31 aa, synthetic construct; identical to SEQ ID NO: 391

SEQ ID NO: 547 - protein, 8 aa, synthetic construct
GAGCVGKS

SEQ ID NO: 548 - protein, 31 aa, synthetic construct; identical to SEQ ID NO: 338

SEQ ID NO: 549 - protein, 8 aa, synthetic construct
GAGDVGKS

SEQ ID NO: 550 - protein, 31 aa, synthetic construct; identical to SEQ ID NO: 345

SEQ ID NO: 551 - protein, 8 aa, synthetic construct
TAGHEEYS

SEQ ID NO: 552 - protein, 5 aa, synthetic construct
GGGGS

SEQ ID NO: 553 - protein, 6 aa, synthetic construct
LLSVGG

SEQ ID NO: 554 - RNA, 61 nt, synthetic construct
  source 1..61: mol_type = other RNA
agtcctccccatcctctccctctgtccctctgtccctctgaccctgcactgtcccagcacc

SEQ ID NO: 555 - RNA, 170 nt, synthetic construct
  source 1..170: mol_type = other RNA
ctcgaggtgtgtggaggacaccctgaaccccccgctttcaaacaagttttcaaattgtttgaggtcaggatttctcaaactgattcctttctttgcatatgagtatttgaaaataaatattttcccagaatataaataaatcatcacatgattattttaactatgctagc

SEQ ID NO: 556 - RNA, 101 nt, synthetic construct
  source 1..101: mol_type = other RNA
aaaaaaaaaaaaaaaaaaaaaaaaaaaaaaaaaaaaaaaaaaaaaaaaaaaaaaaaaaaaaaaaaaaaaaaaaaaaaaaaaaaaaaaaaaaaaaaaaaaaa

SEQ ID NO: 557 - protein, 189 aa, Homo sapiens [sequence omitted]